European Patent Application EP 4 640 055 A1, published October 29, 2025. Title: ISOLATED BACTERIOPHAGE AGAINST XYLELLA FASTIDIOSA. Applicant: BIOLINE AGROSCIENCES FRANCE. The sequence listing filed with the application follows.

SEQUENCE LISTING (35 sequences)

SEQ ID NO: 1 - DNA, 62014 bp, unidentified
  source 1..62014: mol_type = genomic DNA
cctcccgccgctggagcaggtccgggcgcactgggacaagaactttggaggcccgttcgagtggcccaaggtcgaaccgacccaggagcctctgaaggacggcccgaagtcggacaagccgccattctgaggacgcccccatgagcgagacgctggaagcaacgaagcgggagctggagggggcggggatcgcctacacggtggagctgggccggagacactacaaggtccgcttcaccgtgagggggaagcccctgatggtgacgtgctcgcggacttcctccgaccaccgcgcggccctcaacgcccgccttcaggtccggcgggaaatccgccgtgcgctggaattgacctgaaccgctttacttcttcggactgacccactatacttcttcacacgagtcgagaaatgaaccaaccccagacactgacaccgcgattcgagattggaaaggagctgacccatcatgaactacaagaagccttccgccgcatacacgggcacccaatcccgcgcggcgcaaaaccgcaagaagtcgcacgaggacttgctgcgcgaagcccgttgcgattcgagtttgaagtcaatcgccttcgaggctatgcgtgggacgctgacgaggttgagtgaccacgcccgctgggctgctccgcttgccttcgccgtcctgctgctctggggcctcgcgggggcctttgcggactacctggaccgcccggaggttcatatcagctacctgacccgggagtgtgtgcgcgtggtgaacgcggacggctcccccggatcgtgtggagccctcccggaccgctatgagcgagtgtgggtggagtaagattctgtttcaacaaccctgagaaaaggagtcacaacgtgatcatcttccgcaacaagggcgtcattgaccccaagtccatcaccaccttcggggtcagctcgaaggagaaccccggggccatcggcttcttcgggaccggcctcaagtacgccatcgccatcctcctccgcgaaggctgcgacatcaccattcacgccgggaagcgcaagctggagttcggcatcaagcgggatcgcgtccgggtcgatgacttcaacgtggtcacgatgaacaaacgccgtctgggcttcaccacggaggtcggcaagacctgggaattgtggcaagccttccgcgagctgtactgcaacacgatggacgaacgcggcgaagtgttcgaggccgatgaggtcccggaagtcgccgcggacgaaaccgtgattgtggtccggggcgaaaagttcctggatgtctgggcctcccgctctgacatcatcctgtccagcgagcctctggagcgacacgaggccgtccacatccatcccggcccgtcgcacttcgtgtactaccggggcgtgcgagcctaccggctggaccaaccctcgcagttcacctacaacatccagaagaaggtggacctgacggaggatcggaccatcaagtggtcctgggacatcagcgccgccgtccgccgcggcctgtgcgagtcgcagaccgccccgctgatcaagaaggccgtgaccgcgcccaaggggacgttcgagcaccagctggacttcgagggcgtggagccgtccaagcccttcctgtccatcgtctccgaactggcgcgcaacttcgactccagcctgagccggtcggcgctgaaggcgtcccaggtctggatcatggaccagctccacgaggaggcgaccccgatgcgcctgagcgagctggagcggacccggctggagaaggccgcgacgttctgcgagcggctgggcttcgccgtccaggagtacccgatcattgtcagcgagttcctgggcgaggaggtcctgggccgggctcatgagggcaaaatctacatcagcaagcgcaccttgatgatggggaccaagatgctggcagggacgctgattgaggagttcatccacctccgccaccagttgtacgacgaaacccgcaccatgcagaacttcctgatggacaccatcgtgtccttgggcgaacagatcaccggagaaccgctatgagcaagaccaccattcgccttaccggagacgccctgagcgccgcccggattgtccacggcatccaccaacaggctcacgcccagaaggcggagctggaacgtgagtatcaagaacgcctcaccgaactcgggaaggaggcccaggagcagatgagccgggcttggccggggctgatgcgtgccgcagacctcccgctggaggagctgggtgagtgggagctggacgcgagctatctggatgaccacggctgcgccttcctcactaagcgcgaggaggacgcccgcccctccctgggcgacctgctccagtccatgaccgcctcgaagcactgaggagcccgactatgaaaccgctgctgatcttcgtcctcgccctgctgcccctcgccacgcaggcggcaccggaggaccgccccctgtataacgcccaggagacggtccggcgtgcgcagattggcagcaattccccacgcctcgcccctccgtcccgggtcctcccggcggaggtcggggcgaagccggacccggcccgcttcgagcggctggagtgctggcacgatcccgcccgacccctgggcaaccgtattgtttgcgaacctcggagaacaaaatgagcaatgaaacccaagaatccatcacccgctgggctgacgaaaccttcggagtgaagcacccggcggaagtcgccgcccgtatgaacgtggaggtggcggagctggtcgctggcctcgccaccgtcgccgccgtcccggtcgaagatatggacccggagctggtccaggaactccagaaggagtgtgcggacgtgttcatcatgctcgcccaggtcgcggagaagctggacgtggaccttcagaccgtggtgaactacaagatgggggtgaaccgccgccgcaactggaccaagagcccgtccgggaagatgcagcatgttgagacgttcttggagccggggagcgggcttgagatggagctggacaagttctacatcctcagcgactcgggccacttctacactgaccggggcttcgagtccgcggacgccgccctgaactgggcccaatccgcggaggggatcgccgccggagccgaaggagcggtggtgccgaccttccgggccgggggcttcttcgagggccaggacggcgtgaacatctacctgggccgcgagctgcgcgccttctggaaagccaaccccctgaacgaaggagaacccgcatgacgacaacaatccagggcatccaggcccgcctcgggcgcaacccggaggacccccgcaagtaccaggtcacggtcctggtgtatagccaagtccgcccaggcctgaagtcctccacggacatcgaccccggccagtgcgcgaaccagcagcacctcctccagctgatcgggacggcgggggccgcttgcgcggagtacctgggcaacaactacggggacaacatcgaccccgtggccgcgtcccgggacgccatccgcgccttcggggaggagtgccggctgatggcggaactcgccaaggacgtacccgcgaagctgaagcgcctcgaaagcaacgtggcgaagctgtccaacgagaaccaggaacagttgcgccgcctccgctacctcgtggaccatcaggagaagctgctgcccaaggaggtcgcgtggctgaatcagcgcctcggggaactccacggaggtcagctgtgaaagacctggacgaagcggccctggccgttctgttcgaggagtaccggcaacgccttccggtcgcggactgggaggagttcctggtcatcgcccggggcgtccttgcctcggagcgggtccggtgccgagtccagcgccgggagtattttgtggaggactacctggaagccgatctgcgccgccattttgacacgctggcgcatcgtttcggatcgcccgccctggcgattcccggaccgcgaccgctccagctgaaggaactcccgtggtggaggcgctgggcgctgctcgccctcctcccgaagccggatgacgacaaaccctgatcaacacggagacaattgatgatcgagacgaacaacccgggccatggcttcttcggaacctacgccctgaagaagggcgaggaggccgcgcgcaaggcttgggccgtggccttcgaggcaatcgccgccgccgtaccctccgcgaagccggaggaggtccgcaactacctggacagcgtgtacgggcgtcacaccgcggatgaggtcctcagcggcccgtccgtcgcccaccaactccagttccgcgcggcccgcttccgtcgccacttcgcggagattcaacgccaaaccgcccgcggggccttcgaggactgaccatgataccatttgaccaagtcgaagcctacgtgggcgacttcctgagcgaactccacggacggggcctgggcgggaacatcgtgaaggactcccccgcccagctcatctacccggagcgggcgctgtggaccggggaagcgcaccagctcgccttcctgggcgagccgggggactaccgcctggagctgcgccggatcgaaggcgggcactgggaggcgatccgcgaggagcgcgacccggaccgcttcaacctgctgatcatcgacctctgcgtgaaggagggctgacgccatgaaccaagacccgaacaagcgccccaacgggacgtacaagcccaaggcggagcggttgccgcctcaacatttcaactgtcgctcctccctcccgccggtgaaccttgacgcggcgatccacgggggcctccgccttctcgccttcgccctgttccgccaggctatcgtggaggctatcgtggaccagcgcgagacggcccaaggtatcccgaccggcgacggctctgcggcgacctcctgggaggagctggagcgggtcctgggcaaggagacggtggacaggatgagggccggaacttgaaggaggaccggagctgggagctgtgctggatcgtcccgggaggttcccttcaaaccaagaaggtgacgggctacgcccgcgcctgtcaggaggccaagaacctccgattcaagatgcgcaagaccgaaggagtgagaatatggatcatgagcgagttctgagctggctgcggagcctgttcaggcggacgcccgccgccccgccgccggagtcgggaccgatcacctggcccgggatgatggccccgggcttcgaccaacaacccctaccggagaaacaccccttggaacttgatcatgaacagtggggcagcgtggtgaaaaacgacttcatcaggaccttcttgggcgaccgcctggggttcggagtcgcccgccaggtgtatgccctccacggacaaaccgcccttgtggctaaggtcgaaaccaccgcgcagtccttccagaatgtcgcggaatggcagatgtggcacgaggtccaattcaccccctgggcgcgctggttcgccccgtgtcgccgcatcagcccctgtggtatcgtcctgatccaggagcggacgcgacccctgccccatggcgaactgccgaaggagctgcccgacttcttcaccgacctgaagccggagaacttcggcctgatcgacgggcaggtggtgtgtcatgactacgccctccacctcgcctcctcgaactggttgggcaaggcgaagatgaagaaggtgaagaaggacgaatggcgactgcctgacgaagattgacaacccgacagaaacggagaacaaacatggaacatatcgacatgacggacgccgctgctgagttcatcgacaaccaaggcgtggctgacttcgcggacgcgatgcgccgcaagctggagaagaagagggcggagggccggggcggttggcacgaccccgaccagtgtcaactggacaccctcgcggtgatgctgctggatcacctggagaagggcgaccccgtggacatcggcaacttcgccatgatgttgtacaaccgcggcgacggagcggacggtcagccctccgtcctcggggcgaccttccgcgaatggctggatcaccagctcaaggcccgggacatcgtcgcctcgaacctccaagccgctctggacaaggccgcggcccggatcgcggagctggaggggatcgccggacgcctcgaaggcgagcgcaacgaggcccgccggtcgctggacaaggagcgggaggtgttccgcaaggagctgggggcggagcgggacgcccgccgccggtcggagctgaacctggcccgtgcccaagggtacatcgaccgcgtgacggaaggcgaaccgccgctgccgggagtgcgcaacgaggtccatgagcgggtcggacaggtcggggtcagctacatcagcggaccggatcgccgcggaccgcgccttgacctgggcgaacccctcagcgacccctatcaattccgctgatggcccgccggaaaccccgccgcggggagtacgtctgcacctgcggggcctatcggttcccgcaccgcttcggaggcggtcgctgctcgggctacttcatcgccgtggagcagtgggagtcgcactatgggaccggcgactgccgccactgtaactgcctcaaccggacggaggccgtgccctactgtgaagtggtggagggcggcgagtcggtccaggaatgccccgtgtggcaagagtttgtacgattcaatgagatcaaactgaagaaggagaagtgacatgagtgacgacaacacgatggacagcgtgatgattgacctggagacgatggcgaccggccccaacgccggggtcattcaggtcggggcgatcccgttcaacagccgaaccggattggtgaagccggacctgttcgaggtggacgtggacctccacagcgccctgatgctgggcggcgaggtcgatgcctccacggtccagttctggcgggaccggggcggactccagcccaagcgcccgccgaaggcgatgcgctccgcgctgaccgacctcgcccgctggttgggcaagtacccggacctgaagcgggtctgggcccaggggccgtcctttgacgtcgccattcttgagggttactatcgccgggcgggcgtcccgatcccgtggggatactccatgccgcgggacacccgcacagtgtatgacctggcgaaggagcggggctggtcgaagccggaagggacgcaagccgttcacaccagcctggaggactgccgccgccagatcatctgcctcatgagcgccctgaacgtcctccggggcaaccctgaaggagaacccaagattggctgacgaaatcgacttgagcaatgaccgcatcctccacgacacggaccgcgaagtggcccggatcgcggaggccgcggcgaagattccgcccggggagccgggcgactgtgacctgtgtggcgaatggagcgggaggctggtgggaggagtctgtgcgccctgtcgggaccgccacaagttgccgtgaatcgaagaaagttgtatgagggggctttacttcttcgggagcccccactatactttcttcacgttcaacaagaacggcaaccacagaaatggagaacatcatggcccgcaccgcttccttctacatcgaccgcgccaccgcccgcttcgaggctggtttcacctccaaggccgctcaacaagaagccctccgcgacctcaacagcgccttcgagctgctgaagcgcgacatcaccggcctggtcctggacatcgaccgggacgcccgcaccgcggatcatgatgacgtgtactggaacctggccgactacccccacaactggaaggccaagcactccgccctcgccctccgcgtgttcccggaagtcgccccgaccgtcgcccagatcgaagccctggtgaccttccgcgccgccgtgaaggccgccccggtggtgaaggtcgaacgcgccagcgacaccgccaagatcgaagccgtgaccaagtcggtccgcgacctgatggagctgcgccaggagcagtacaacaacgccctccgcctccacgacatcttcggcgggctcccggtccatgccaacgtccactacgtcaccaaccagcacggcaccaccttcctccgcgccttctactacctgaacggcgagctgaccccgctgggcatcatcatcgccgccgcggaggcgaaggcccgggaagccgaaggcaagtgagacgaagcgggagggctccggccctccccacccaagaaaaggagcccgatcatgtacaacatccacaaccgcaccctgaacccctccaccttcgtccccaccctgttcatcggagtcggggagctgggctgcttcttcaccctccgggagacgtacctgcacgccgtcccgggtcccggccccatgggcaacgcggtggtgaacggtgtgtatcagggcagcttcgaggtccgcagcagccacgtgaagaacctgagccaggaccctgacgaagccttcgagaaggcccaagaagcctcggagcgcatgggcctgaagctcacgacctcccgcgactccctgcgcgaggaaatgaacgcgattcaccgcgccaacgccgcggagctggagcgccgggagcgcgagcggaaggagcgcgaggaccgctgggccgcggaacgggccgcggaggaggaggagaagcgccagaccatcctgggcggcaagttcgccttcggaccctacgcgggcaaggagttccacgaggccccgcggggctacatcagctggttgatcgacaccctcccggacttcgaggaagggggcctgatgcgcctgaccgcccaggaggtcgcccgccgggtcccgcacctcgccctgccgaagccgaagcccgacctgtacgtgggcgagccgaagaagcgcatgaccttcgacgtgaccgtggttcgccgctacaccttcgcccgggacgcctggaacggctatggcatcgagacggtccacatcatcacgatgatcgaccgcgcgaccggggcctgcctcgtgtcgaagtccggggccttctacgcggaggaaggcgaggagctgaagatcaaggccaccgtgaaggagcacgcggagtaccgcggccaggcccaaaccgttgtccagcgaatcgcggtgatggaggactgactcatgcgccccaacctactcaaagccctccgcggaatgagcgaggcggagctgtacgcagccctgtaccaggaccccctcaccggggtcctgaaccgccgcgccttcgatgaagtccagtcggacgctatcgcgctggttgacctggactcgctgaagtgggtcaacgatacccacggccaccgcgccggggatcaagccattcaggagttggcggtgcggttggtcctcgccttcgggcctgacgccgtgtttcggatcgcgggcgatgagttcgtggtggtcaacgggaaccgggaggagctggccgaccgcctggagaaggtccgcgccgcgttccccggcttcagctttgggacgggcgcgacgttgtgcgaggcggaccgcgacctgagacacgacaaagcggagcgggagaagtccggcgaccgggcggcgaggggcgaacgaccgaagtgggtgccttgaacgcccggcggggctttacttcttcgggtcccgccactatactttcttcacctcaatcagaaatggagtaccccaacatgagcaagattaccgccacccgcatcgacaacgacgaacagcgcctcgaaatcctcccgaccttctttggcgcagacttcctccgggtcgaaatggccctgtacagccacctccagaagatgtgcgaggagtacaacggcgcgtactggtacatgtacaagctgtccaacggcgcgatgtacctggccccggcgattgagaaccggaagctgcgactgaccgtggacaccaatggctactcgggcgaggtcagcggggacgccgcgggcctgatcacctgtctgttcgtgttcaacgccctctgctggaagtacccccagcgcgaggacttcgtggacctgttctacaagctgcgtgacttcgccttcgaccacccggaggctgaggaaatcatcgccgccatcgactgaccaaccccctcggggcggatcggttccgccccgaacttcccagaaaaggagcaacaccatgaccaagaccacccccaagaccaacctcctggaggagaccatcaaccaaggtcgccaggacgtgaccgcccgccgcgtcctgtccctgggcgacttcaaggtgcgcctcacgatcaagtccgacagctacaagttccagtccttcgcccgggcggaagtctggaacccggcgaccctgagctggaaccaggtccactccatccactacgcggaaatggcgaccccggagggcctgtgctaccacccgaacaagtccggcctgaagatcacccacttcacccgcgacttcgaccgcctgctgacgatggtcaagcagatcatcctgtaaccttgtagaaaaggagcccgccatggccaacatgagctactgccgttgggagaacaccctcaacgacctccgcgactgcgcggaacacgtgaacgaccccctgggcggatcggaagcccgcgcccgggcgtccctcctcgaactcgccgcggacatgctggaggaggtcggggtgaccatcgaccgccgcgagctggacgaagccctgagcaacgccccgggaggtgaaggatgagcggacgctacaaggtcctggtcgggtcccaatccggccactgctgcttcgactacaccgtggtggacaccctcaagccccaccccgtgtatgcttcgcaaggtctgttcgatgcgatctgcgagacgttcagcgaggaggaagcccacgcggtcgcccgcgccctgaacgccgcgaccacgaaccaggcgaccctcgcccgggccgctcgcctgttcgaggaggccctgcccaagttcaactggggcgcgagcgccctggacgccaacgcgatccagctgctcaacgaggtcccgggcgaagtccgcgcggccctgaaggcttgcgccctgtgcggaggggaaggccacacggccccgaactgcccctgggcgaaggagggcggagcatgacccccgcaaaggctgacgccctgatccaggagttcatcgacctgggcgaacagatgaagcggctgaaggaccgccgggcgaagatcgcccaacagttcgccccgggacggacggaaggcgaccgcctggccctgtacgtcgccgggcggggctactcctcccgcttcgacgcggccctgctgcgccggtacgtgcccgccgccacgttggacctctgccgcgtgacgacctacaagaacggctccgcccgcgtggtgccgaagtcgaaaccaagacccaagaaggagaagcgcgcatgaagcggggaatctaccgcgtcccgatcccgcacctgatcggcaagaccgcgctgctgcgcgaggcgacccacggccatgtcgtggcgcagttcgatgactggagcctgacccggagcggcgacccgatcccagcggagaagcccgaaggcccgcccgcggacgccctgggctacggctggcacgccttcccggcggaggacttcgaggagaaccggacctgcccgacctgcgaggcgaccggctttcaacaaagcacgctgggtcccgaccgctgcaccttctgcgatgggacggaaggcgggaacccgccggaggaggacgcatgaacacgcccaacaccccgcccgaccgccgcgtgcggtccatgacctcctccgtgggcacgacccgcgacggctacctggtccgccaagtggttgtcgagtgcgaggacggcacgctgtggcgactctgcgacaacgaagccgggactgatcactgggtccggctcccggcgatcccggggaggtgagacgatggtgctggctgaaatcgagtcgcgcatcagcggcattccttgtataatcgccgtcacctactgggaaccctacgtgcccgcgaaggtgagcggaccccctgaacactgctacccggcggaaggcggatgcggtgaatgggaagtccgcgaccgccgcggacgccccgcgccctggctggagcgcaagatgacggaggcggaccgcgagcggattgaccaacaagtgttcgactacatggaggaccgctgatgaagcaacgcctgctcaagcgagcccaagaccgcatctgccgccgcctccgcgcccgcttcacgatggtgaagccggagccggtccaaggcatgttcaacttccgctgccacgagaactgcgtggagtacgtccgccgccacccggaggagaagctggccgtggtggagacgatctacattgacggcggcgagcccatcctacactacctggtccacgaccccgccgcgggccgctacctcgaagtgaccctgggctggcgggcggagcacctggaatactacgttgtcaggaccctacacccggacgatcaccaccacatcctcagcgagttccaacgctccctggacgattggacagaggagtacgtgggctggttcggtcggaaggtcctgggcatcacgagggtcctgtgatgaagcacctacacctcgaacgcctggaccaagcccttcaacacgccgtcgcggacggatgcgacccggcggacctcctcgcggaactcgccgcccgacacctgatgagcgatgaggcggacccggcccatgtcaacggcatcgccttcgcggaacggttcaacgccgccctcgcggcgaaggccggaggaggcgggacgtgacctgcatgcgcatcccgggcggcatcgtctgcctgtcgcccttcttccggctccgcctcgcggacggctcctgcgtgttcatggagtggcacaactactgcgggccaaccttcttccgcgaccgggcggcacgccgcatgattgacgagtggtgggacaaccccgcgatctgcgccgccctggactggttcatccaacgagggaagcgggcctgaccacccctcacgatcaatgccccgccgggcggcaatggtgccgacttcactacaggaggccgaaggctgcgggaaaaccggcggggctccctcctccttctccacttcgaccgggtgcgcttgggttacgggagtgcgcttgggttcggctccgaaaaagtatgaagcaaggcgtggcgggaagtcaagcccgtctggggttcccgcaccttgcgcttaggttacttgggattcttacctgaaataaattcgcccgacaaatcgacccggcggaccggcccaggagaatccttgttgaggctttctggtgtccgaagggctcccagggggttaaggtaagtaagttaagtaagttaagtatctatctatctatctatctataaagggctgttttatatggcctttttgcccgcttgactttttacttcttcggacgtggaagtgaagcgcgacccctcgaacctaagcggaggacgctgcctgcctgcttgggcaatccgctgccacacgctcctcgtgcctcccccgcgggcgagcgcgactcacccttggctaatgtacaagctcacgctatactcgcggcgaggatgtccttgggcgtgaggccggggacggatcgccgcgtgatgcgcgattgacgaacagtacacaccgaagggggagcgtgatgcacccgattgagaaactgaagccgaagccgatggtgcccttcacctcggaccgcaaggagcagtacctggagttgttccgcacgcatcccgacctgggtgggcggaagtacctgtgcgcggaggccgtgggcgtctccggctccaccatcgactatcatgtcaagaatgacccggagtttgcccaggctctggaggacgcccgccaagcgtggattgatgagcacctgttcagcgcggccctgaagcgggcgcgggacggcgtggagcgcccgatcatcggcgggaagttcaaggacgaaatcatcacctatgagcgggtgtacagcgattcgctgatggccatgatgctccgcgcccaccgtgcggagttcaaggacgggaaggacgcggccagcatgaccgcctcgggcaccggcggggtgctgatcgtcccgggggctccggccacgatcaacgactggcagaaccagtttggggacctcgcccgcgggaccgtgggccgtccgaccggggagggcagctgatgttcgcccagaccgaagtgagcaaggcggtcgccatcgccgcccgcccggactacccgattgagtggcgcgaggcggagcccggcgagctgcggggctactacgtggacccggagacggggaaggagtcggaggcgacctggtgcccgcagtacgggtcgcagctcgccttcctcatggcgcacccgatcttcgaggtgctgtatgaggggacgcgcggcccgggtaagaccgactgcctgctgatggacttcctccagcacgtggggaagggctacgggtcggagtggcgcggcatcttgttccgtcagacctacccccagctgtcggacgtgatcaacaaaaccaacaagtggttcaagcgcatcttcccgggggccaagtacaacaaggtggagcacaagtggaccttcccggacggcgaggagctgctgctgcgtcacatgaagtcgccggaggattattggaactaccacggccacgcatacccgtggattggctgggaagaactctgcaactgggccgatgacaagtgctacaccgtcatgatgtcctgctgccgctccacgaagccggggatgccccgctgctaccgggcgaccaccaacccctacggccccggccacaactgggtcaaggcccgcttccgcctcccccacatgcgcggtcgggtgatcctggacgcgatgcgagacggcgagcgcgaaccgccccgggtcgccattcacgggtccatctatgagaaccaaatcctgctccacgctgacccggagtacatcagcaagattcgagccgcggcccggaacccctccgaactcgccgcctggctccacggctcctgggacatcatcgcgggtgggatgtttgacgacatctaccgcggggacgtacacgtggtgccctccgtcccgttgtcggtgatcccgaagcggtggaagattgaccgcagcttcgactggggcagctccaagcccttcgccgtcctgtggtgggcggagtcgaatggggagccgttcgagtggaatggccgcgtgtacgggaaggtgcggggcgatctgtacctgatccaggagtggtacggctggaacggaacgcgcaacgagggcgtccgcatgctcgcctcggaggtcgcccaaggggtgaaggaccgggaggaggactgggcgctggaaggtcgggtcaagcccggccccgctgactcctccatcttcgacgtggagaacggcaacagcatcgccgtggacatggagaagaagggcgtgcgctggacgcccgcggacaagggcccaggctcgcgcaagcagggctgggagcaaatccgcaagctgctcaagggggcgttgcctccggcgggcgggggaccgcgcgaggtccctgggctgttcatcttcgactggtgtcagcagaccatcgagacggtccctgtgctgccccgcgatgacaaggacctggatgacgtgaacacggaggcggaggaccacattggtgacgcgatccgctaccgcgtgcgcaagaagctgcgtggcgtcaagcagggcaacatgtaatacaacttgccgggtcctcgccttcgggcgagaatccgcgaaccaggagaaccgaccatggccgacaaagacccaaagagccccgccacgaccagcggggcgtatgaccagatgctcccgcgctggcacgtcatcgagacgctgctgggcgggaccgaagcaatgcgcgaggcgggcgagacgtacctgccccgccaccaggaggagacggacacgggctatcaggagcgcctggcctccgccgtcctcctcaacatggtcgaacagacgctggacaccctgagcggcaagcccttcagcgagccgatcaagctcaacgaggacgtgcccaaggcgattgaggagacgatcctgcctgacgtggacctccaggggaacaacctggacgtgttcgcccgtcagtggttccgcgaaggcatggccaaggccctctgccacgtcctcatcgacatgccccgcccggccccgcgggaggacggccaaccccggaccctggcggatgaccgccgggagggcctgcgcccgtactgggtgatgatcaagccggagtgcctgctgttcgcccggtcggaggtgatcaacggggtcgaagtcctccagcacgtccgcatcatcgaacattacatggagcaggacggcttcgcggaggtctgcaagcgccgcatccgcgtcctggagccgggccttgtccagctctgggagccggtgaagaagtccaacgcccagaaggaggagtgggcgctggtggatgagtgggcgacggggttgaactacgtcccgctggtcaccttctacgcggaccgccaaggcttcatgatgggcaagcctccgctcctggacctggctcacctcaacgtggctcactggcagtccgcctccgaccaacgccacatcctcaccgtctcccgcttcccgatcctcgcctgctcgggggcgtccggggaggactcggacccggtggtggtcgggccgaacaaggtgctgtacaacccggacccgcaggggcggttctactacgtggagcacaccggccaagccatcgccgcgggccgcacggacctcaaggaccttgaggagcagatggcgggctatggcgcggagttcctgaagcgcaagaccggcgggcagacggcgaccgcccgggcgctggacagtgcggaggcgaccagcgacctgagcgcgatgactgggctgttcgaggacgccctggcccaggccctggacatcaccgcggactggctccgcctcgggccgaacggcggcaccgtggagctggtgaaggactatgacctggaggaaatggacgccccgggccttcaggccctccaagtcgcacgcgagaagcgcgacatcagccgcaagacctacctgaacggcctccgcctgcgcggggtcctcccggaggacttcgatgaggatgaggactgggaggagctgatggaggaaatcagcgaggcgatgggccgcgctggcttggacctggacccggcccagaagaacccgcccgaaggtggggagggtgagggtgagggcgaaggcgaaggcgagggcggcgaaggcggagaaggcggtggaaatccgggaggcgagtcatgaacgtctggcacttcttggggctttggctcctcctgagcatcgtcctcgccccgttgatcgggcgttgtatccacttcggcatgaacggacccaaagaaatggagaagcgggatgcccacattcaatgaggagtaccgggacgccgcgctgcgtcaccaaatcgacctgcgccgctacaccgcgggcgtcaccaagcgggtcgcccggctcctggaggaggcggaccgcgacctgaccgaacgcctgcgcacccggctcgcccgcttcgagggccgtgacctggacttcaccggcgaacgctggaaggccctgctcacggacatccgcggagcccgggccgcggccctcgcggagtacaagaccctggtgcgggacgaactcgggcagctcgccgtcctcgaaggccaggccgaaatcgacctgctgcagtcctccatcacgattgaggtgggcttcatggcggtgaacgcggaccagctccgggccatcgccacctcccgcccgttccagggccggttcctccgggactggttcagcaccctggaggcggtggaccagcagcggctgaccacggctcttcagctcgggatgacgaacggggagcccattgacgacatcgtgcggcgggtggtcgggacgcgcaagaacgcctatgcggacggcatcctgtcgatgacccggcgggacgcccaggggatcgtccgcaccgcggtgaaccacgtgtccaacaccgcgcggggctacgtctgggacgccaacagcgacatcatcacggcgaaggtctgggtgagcacgctggacggtcggaccacggctgtatgccgcgcccgggacggccacgggagccccgtgggcgacaatgagctgcccgcggacatccccctgctccagcccaaggacgcgaagcccccggcccacttcaactgccggtcggtgatggtcgcctacatcgacggcgtgggccttctgggcaatcgcccgaccgtgacggacacccggacccgcgccaagcgtgaaatcgacttccgccggatggcgaaggagcagggcaagccgatccaggacatcaggaaggcttgggccgcggagaacgtgggccgggttccggcggcgaccacatatcaggacttcttgaagcgccagcccgcctccttccaggatgaggtcctgggcaagaccaaggccaagctgttccgggaaggcgggctgaacgtggatcaatttgtggatcgggccggcaacgagctgaccctgtcccaactcgcggagcgcaagccggacgccttccgcaaggctggccttgaccctgaaaagttctgaggctacaatatgaaccgtgcgtgaggcacaacactggcgggtgatccgccgacaatgaggatacaattatggactttgaattcactccggtcgattccatcgacaaggtcccggaacagttccggggaatctacaagcagggcgatgatggcaagttcgtcccggacgaagcccacaaggggatcgtggaggccgtgactggcctgaaccgctccctcaaggctgctcgtgcggaggcgaaggccaagacctccgtggacctgaccccgctggctgacttcggtgcgacgccggaggaaatcaaggccaacatcaccgcgaagctgaccgaactccagaatgaactggccaagggcggcgaagccaagctgaacctggacaaggttcgccaggagctggccgatgcgcacgcgaaggacctgaagaaggccggagcccgcgccgaagccctccagaaccagctgtatgggctcctggtcgagaacgccgccactgccgccgttgcggagctgaagggcgtcccggaactcctgctgccattcatcaagaaccaggtcaaggtggtcgagcaggacggcgaattcaaggtgttcgtggtcgatgcccagggtgaccagcgttactcgggcgtgaccggccagcccatgaccatccgcgagctggtcagcgaaatgaaggccaacgagaagtatggccgcctgttcgagtcggaagccccggcgggcggcggcatgcctccgcgtggtggtcagacgcctccgcgccagcagggcaaggtcctgaccgccaacgaaaagatcgcccagggcctcgccaagggtcagttcaaggcgggccgcggtcgggcgtgacggatcggggaggcccccaagtttggccagggggcttcccttttccgcaacttggtactatactgacgtcacttttggttgtatagccagaggcgaaggcccacaggagtgattccgcgggccgcgacggaacaccgggtgatccggcacggctgaaaaccgcttgagtcatcaacttccgaaggagggccaatcatggcttctgttacccttgccgaaagcgccaagctggcccaggacgaactggttgctggcgtgatcgaaaacatcatcaccgtcaaccgcatgttcgacgtgctgcccttcgactccatcgaaggcaacagcctcgcgtacaaccgcgagaacgtccttggcgacgtcatcatggccggtgtcggcacgaccttctccggcgcgggtgctggtaaggccgctgcgaccttcaccaaggtcaactccaacctcaccaccatcatgggtgacgccgaagtgaacggcctgatccaggctacccgctccggcgacggcaacgaccagaccgctgtccagatcgcctccaaggcgaagtccgctggccgcaagtaccaggaccagctgatcaacggcaacggcgcgggcaacgagttcgcgggcctgatccagctctgcgcctcgggccagaaggccacgaccggcgcgaccggctccgccatcagcttcgccatcctggatgagctgatggacctcgtggtggacaaggacggccaggtggactacatcaccatgcatgcgcgtaccctgcgcagctacaaggcgctgctccgcgccctgggtggtgcgtccatcaacgaggttgtcgagctgcccagcggcgcggaggtcccggcctactcgggcaccccgatcttccgcaacgactacatcccgaccaaccagaccaagggcggcaccactggttgcaccaccatcttcgcgggtacgctggatgatggttcgcgcacccacggcatcgccggtctgaccgcgacccaggccgcgggcatccaggttgtggacgtgggcgagtcggaggactctgacgaacacatctggcgcgtcaagtggtactgcggcctggcgctgttcagcgagaagggcctggcctgcgctgacggcatcaccaactaaggcggcacccgccctccggggagggctctgccccgtagtacccgaagggcgggccggtctgagactggtccgcccttttgttttgaacgcactcaggagacgctatcatgcccgcttaccttgtaaccttggaccggaacaagtccggccacacccttgtccatggcgctgacgccatggttgtgttcgccgcctccgctactgccgccaagcaagctgccgcggcgaagtacgaaggcgacggcctggcctggctgaacgattcgaccgccaccgaaatcgttgccggcaccgactggtccggctggaccttccgcgtggcgatcctcggaggcttcggcaccggcggagacgaaccgcgcaccgtcgctgtcgtgggcgatgcgaccgacaacaccgtggacgaaatcgccgcggccctcgtggtggcgctgaacgccctggacgggatcgccaacgccgcctacaacgcgaccacgaacacgctgaccgtcgccgcggctgcggacgccctgggcgaccagaagctggaagtgtcgatcatccccccgggcggttcggcctccatcgcctccctcgtgggcacgatcacggatggcggagttgccgctgccgacctgaccgtggtgctcccggcggacaacgccgtgatcccgaacgtcctggcccccgtcgcccaggtctaacaccaaccccggagaactgtacaaatgtccaccatcatccaaacaacctttgtcctgaccggacccctggcgggccgcacgatccgcctgggcagtcagccctacccgttcgacaagggccgcttgaccatcaccgctccggcggaggaggtcgccctgcacgcccgcttcctcgaacgcaactggcaggcttacccggaaggacacccggccctgaaggaggtgcccgatggccagcgtgatcttcaagaaggcccccagccggacggccaacagccggtacacggcgacgttcagcccaacggggacgggactgaagccggtgacgcggcacctgtcagcggcggaggtgtcgaagccgaagccgggcaagccgggggtgtacccgatggggacggacaaccggaggtcctgaccgatccggcgaaggagccgaccctggagctgaacaccaagctccagaaggcggtcctgggcctggacccggcggatgacactcactggaccaaggacggaaagcccgcgatgaccgccgtggagaagctgtatggctccgccggcatcacccgcgctgacgtggaagccgtcgccccgggccatacccgcgacaaggcgaaggccgctcagtaacccaaccaactccgaaggagaagcatcatggcgaaatccggcaccaccaaggcaaccgcctcgaagatggtcaatgcctcgaagtctggcgtgcgtcacggccagaactcgaagaacgtggtcatgggcggcaagtccgctccggctccgtccggccccaccgccccgatcaagggcatggacaagggcggggtctgacccgtgttcggcttcccctcctccaaggtctgggctgcggcgggcgtcttgctcgccgtcgccttgatcgccctcgcgggctacggctacggctacggctccgggaaggcggacgcgaccgcggaggcggcggaggccatggacaaatacaaggaggaggtccgcgcccgggaacgggagcaggaacgcctcctggctgaggccaacgacaagaaccgtgaacaggagaaagcccatgaacagcgtgtcgcagacctccgggcggagttcgcccaacagcaagcggacgcccgggcgcgggatgagcgcactattgctgatctgcggtctggcaatcagcggctgcgcctccaagtctcctcttgtggtgcggcccgatccggtgcggctgagtccgcccccggcggagctgatggagccggaacagccgaacttgcgccagagacttcagcagctctctggggaatcgccgcagacggcgaccgggccatcaggaaactgaccgcccttcaggcttgggcgcggtccgccgtccagctgtgtaccctaccgcaaccggagaaccaacaatgaacatcgccgtcacccgcttcctcgcccgactgcgcaagcgcctcgcccccttcctggacctcacggcctgggtcctgctcatcgccagcatcgtcccgttgctgctgatcgacccggccatggtcgtgaccctcgcgcagtggacagcgtttgccctcgcgctggcggggatcaccgttgtgatcacccgtgtggtactaccccaggtgaacctatcggaatggctcgcgcgtgcccgggagggctccgtggccgggggcctcgtggtcctcgccgtcgccctgactatctgcttcaccttcttgggattggtgctatgggcaaaagcctgattcacttcgccttcgcggtcctctgctgggccttcggctccgtcgccctcgcccaggacgcccgcaccttcgtcccttcgggggcgaaggtgtacgcgccagtgctagtcgagaagcagcgggaggtctggccgcaagccccggagccctggaccctcgccggtctggtggagcaggaaagctgtatcagcctgactcactcccgctgctggaacccgcgggcggagctgcgcacccctcgtgaatacggcttcggcttcggtcaggtcacggtcgcctatcgcccggacggctccgaacgcatgaacgtgttcaacgaactgcgcaacacccacgcctccctccgcgactggacctgggagaaccgctatgacccgggcttccagctcacggccatcgtggaaatgaaccggagcctgtggcggaggatcgccgcgaacccgggcgcgacggtcacggaccagtgggccttcgtcctgtccagctacaacggcggggcggcgggcgtcctacaggatcgccgcctgtgctcgaacacccgcggatgcgacccggcccgttggtttgggcacgtagaacgcaccagcctcaagtcccgcgtccctcagcccgggtatgggaaccggagctggtatgagatcaaccggagccacgtgcggaacgtcctgacgatccgccgggccaaatatcaagccttctggaggacgtgatggccttgatcgtccaagacaacacgggagccgtcgccggggcgaacgcctacatcagcgtggaggagttcaagacctaccacaccgaccggggcaactccttcgcgggctccacggacccccagattgaggccgcgatcatccgcgcgaccgactacctggaccagcggttcaacttcgtgggcaagaagcggctgggccgcgaccagaccacggaatggccccggacggacgcctgggaccgtgaccgctactacatcaacgacatcccgccggaggtgaaggaagcctgctgtgagtacgccttgcgcgccctcgccgcggagctgaaccccgacccggagcggaacgcctcgggcgtggcggtcctgtcgaagtcggaagcggtcggacccatcagcgagtccgtcaccttcgtgggcggggccgtgttccagctgcccaaatacccggcggcggaccagaagctggtccgcgcgggccttgtccgctccggcggtacgttgctgcgggggtgatccatggcacggtttgactccgctatcgctctggccaagaagctgatcaagaagaacggccaggccgtgaccctccggggcttcaccgccggggccgctcccgatccgacgaagccgtggaagccgggcggcaacgtcgcggcggaccagcccattgaggcggtgttcctggactatgagcaacgctacatcgacggccagacgatccgcatgggcgaccagcgcgtgttcatgcctgcggagggtctggcggctccgccggaggtcgaaggcttggtgctgcggggcctggaggtctggaaggtcatcgccgtgaaaccgctgaacccgaacgggcaagcgatcatgtatgaattgcaggtgcgccaatgaccctcccgacctttgacagcgcccgcgacgaaatccttgggctgttcaacacgaagtggaccacggacaccccggccctcaacggcggggctccgatccgcgtggaatggcccggggtggacgcgggcgaccctccgcccgcggacaagccctatgcccgaatcacgttgcgtcacactatttcgcggcaggcgaccttcggaccaaccggcggtcgccgctttacccgtcccggactgatcacggtacaagttttcacaccgctgtccgggggacaaggcttgtctcttgctgaaaaatgcgcgataatcgcccgggacgccttcgaggggcgaggcaccgcgagcggcatttggttccgcaacgcacgcatccaggagattggcccggacggcgcgtggtatcagatgaacgtggtggtggagttcgagtatgacgaactgcgatgaaccccttgccacttgaattgaggagttacaaccatggctaacaagattgactcgaacgtcaccggcctccgctatgcggaggaggacacgatcaagaacctgcccgtgtcgccggtgtggtatccgctggagcccaacggctacaatgactttggtggtcagctgaccacggtcgcccggaaccccatcaacccgtcccgccagcgcaagaagggcgtgaccacggacctggacgcctcgggcggtttcggtcaggacctgacccagaacaacctgacccgcctgcttcagggcttcttcttcgcggacatccgcgagaaggccagcaacatcccgaccaacggaaccgccgtgcccttctccggcgtgacgggcaccagcaagacctacaccctgggctctggcacggtggggtcgcagttcctcgccggtgatctggtcctcgcctcgggcttcaaccaggcctcgaacaacggcttgaagaacgtcgccagctccaccgccgtgaccgtggtggtgactcaaaccgcagtggacgagacgcccccggcgaccgcgaagctgatcaaggtcggtttccagttcggctccgctgaaatgaacatcgacgtgtcgggcagctatccgcgcctggtccgcggctcgggcacgaaggacctgacgaccctgggcctgatcccgggcgagtgggtgttcatcggcggggacgcgacggctaccaaattcaccaacgccgccaacaacggcttcgcccgcgtccgggcggtcgctgccgcctacatcgagtttgacaagaccgccggcaccatggtggctgagacgggcacgggcaagaccatccggctgttctacggcaacgtgatcaagaacgagcgggacgcgaacctgatcaagcgccgcacctaccagctcgaacgtaccctgggccaggacgcgaacggcaccatgtcggagtacctggtgggagcggtcccgaatgaactgagcctccagattcgccaggccgacaaggtcacggttgatctgagcttcgtggcgaccgacaacgaacagcgcgacggctccgcgggcgtgaagtcgggcacccgtcccgacctcgtggatgcaccggccttcaacacctcctcggacttcagccggatcaagatgcacctgctgaccgcgggcaactcgaaccccactgcgctgttcgccttcctgacggagctgacgctgacgatcaacaacaacgtctcgcccaacaaggcggtcgctgtcctcggggccttcgacgtttccgcgggcaccttccaggtgtcgggcaacgtcacggcctacttcgcggacatcgcggcagtccaggcggtgcgcaacaactcggacgtgacgctggacttcgccttggtgaagaacaacgccggtctggtgtgggacatcccgctgctcgccctgggcgacggacgcctgaacgtggagcaggaccagccgatcaccctgcccctgtcggtggacgcggcggaaagcgcggcgggttacaccctgctgctcaatgaattcccttaccttccgaacgcggctgacgtataatcaacggagcccggggagggctccggccctcccttccctcaccctacgtggagaaacagagaatgagcctgtacaaactgttcaagaccaacgagaacctggaaacggacggcatctggctggagtacggccaaacggcggacggcaagccgattcgcatcaagatcgcgcgtgccgggggccacaacgtcgccttctcgaaggcgctggagaaggccacccgcccgtacaagaaggccatccagaccgggatgctggacaacaagaccgcggaccgcctgtacaaggaagtgttcgcggagacggtggtgctggattggatcaacgtggaaggcccggacggccagccgatggacttcaacaaggagaacgtcctgaagctgttcgaggacctgccggacctgttcgtggacctccgcgagcagtccgccaacgtggcgctgttccgcgatgaggtacgggagacggacctgggaaactctgggaagtcctctgctacggcttcgagcaaggcccagtagagcagaagatcatcgagcagtgtatgcggttcgggatgcccttgcccgaccgcatacagaacgccccggagttgacccttggttcggagctgtactacatcggatttttggacctgacgtcatgtaggcaaatcggcacgggcctgggacctatcccattgttggccatactggagtattgtatgatcaacgggatcgagggcgagcagcaggaggactttgtttggttcatccagcgacttgaccagaagtatctacagtggagcgcagcccgtgccaagtctaagtgagttcagccgacgcattaccctccggggccgaaaggtcgcggagggcgctgacgcgctcactcgcaaggtcgccctcgccgcggatcaagccgtggtgtctgggacgcccgtggacacgggccgcgcccgatccaactggatcgccgcgattggctccgccccctcctccgtgattgatgcttactcgcccggcgaggcgggcagcactgaagccgccaacactcaggccgcaatcgaccaagctgaatcggtcattcgcgggtacaattacggggaggagattcacatcaccaacaacctcccgtacatccaacgactgaatgacgggtattccgcccaagccccggcgaacttcgtggaacaggcggtgctcgaagccgtccaggttgtacagttcggaagggttgttgacggggacccggggagctgacggtggccgaagaacgcattgacatagtcatcactgaacgaggttcgcgtgtcgttcagcgaaacctggaggacatcggcaagtccgggcgaggagccgcgggcggggtggacttcctcaagaacgccctggcctccctgggcgcgtacctgtctgcgcgcgaactcgtgcgcctgctggacacctacaccaacctccagaaccgactccgggcgacgggccttgaagcccagaacctcggggcggtgtatcggtcgctgcttgacgtctcgaactccacccgccagtccctggagggtacggtggagacgtacagccgactggccaacagcgcgaaggacctgggcctgtcgcagcaggagctgatcgacttcacgaagtcgctgaaccaagccatcgccctgtccggcgcgagcgcgggcgaggctcaagctggtatgatccagctggcccagggcctcgcctcgggcgtcctccgcggcgatgaactgaactccgtcctggagcagctgccgaccgtcgcagacgtgatcgccaagcagctgaacgtgacccgcggcgaactccggcagatgggtcaggatggcaaaatcagcgctgacatcatcttcgacgccttcaagaacgcccggacggagctggaggaacggtttgccaagtccgtccccaccatcggccagtccttccaagtccttcagaacaacgtggtggacctggttggtaagttcgatgaggcgaccggcgcgagcgagctgctgtccaaggcgatcatgttcatcagcaataacctggacaccatcgccaaggtcctcctgtcggtgggcgcgggcttcgctatcgtcgccgggggcgcggctgcgttcaacgcggtccgcaccgcggtgatcgccctcaacgcggccatcgccgcgaaccccttgggcgcattcctgatcgtcctcacctccgtgatcaccgccctgaccctgttccgggacgaaatcaagctggggattgacgacacgaccactctgggcgatctgatgcgcgccgcctgggaggacattggcccgatcgtcaccggcctcgccaatacggtcggggagttcttcaactggctgaccggctccgcggcgacggcctatgagaacatgaccgaccaggccggggccagcgtacagaaccaggaagcctggtggttgaagctggtccgcaccgtcctccaggtgttcgacatgattggcgggacgatccggggcgtgatgcgcggggtcctcaatgtcgtgggctccgtcatcgacgccctcatgaacaacttccgccagctcgggaacgccctgaaggccgcagtggaccttgatgtggacggactgaaggccgcggtgaccagcaacctcgaaggttggaaggccgtgggcgccaacatcgggacgaactttgaggaaggattccgccaggaagtcctcgcccaatccgaaagcgggctggaggcgatgctggacagctggatcgaacgcgcccgcgacatttccaaggagcgggtcgccgcggctcaagtcgagacgccgaatctgggtggtgggggcggtcgccggacctccgggaaaggcgatgaggaggcggccaaggccctcaagaaacttcaggacgaactcaaccaactggtcgggtcctatgaccgtgtctgggcggctcagcaggagtacgccaacgccctcgccttgctcgacaaagcggagcgcgcgggcctgatcaccgcggagcgcaaggcccaggtcctggcgctgatcgaggagcagctgaaggacgccctggacccgatgggcgcgatcaaccgccagctggaggaggagcgcgagctgctgcgcctcacctcggagcagcgcgaggtcgaacagcagttgcgctacatcgaacaggacctgcgctatcagggcatcatcctcggggaccaggagctgaagcagctccgcgagaagctgaccctgattcaggcggaaacccgggcggcggaaacccgcaaccaggtccttcaggctatcctcggaccccagcaggagttcaccgcccagctcacggcgatcaatgagttgctggccgcgggggcgatcacgcaggcccaggcaaaccagttcctggtggagtccaacgcggaccttctcgcgggtacggtcgaagcccagcaggcgatgttgtcgcagtatgagcagatgtacgcgcggattgatgagatgcggcaagccgacctcatcagcgagcagaccgcccagcaattgaaggctcgggtccaggcacagatcactgagcagaacctgtccacccagcgcaacttcttctccaccctgtccgggctgtcccggtcggagaacaagaagctggcggccatcggtaaggccgcggctatcaccaccgcgaccatcgacggcgtgctggcggttcagaaggccctcgcctccgctccgcccccggccaactacgccctcgcggcggcgaccggcgcggtggcggcggcgaacgtcgcccagatcatcgcccagacgccgggctttgccttcggcggcgacttcaccgtgggcgggacgggcgggacggactcgcagctggtcgccttccgtgctacgcctggcgaacaggtgtctgtccgtactccgacccaggagcgggacgaagcgcgtcagggcggtggcgaggggcagcagggcggtgggtccgcgatccgggttgtgaacgtgatcgacccgaacctgatgcaggactacctgaccagctcctcgggcgagcgggtcctgctgaacgtaattcaacgcaacgctggcgcggtccgccaggttgtgaacaacggctgaggatgagacatggcacacgaaatcggaaccgcgacgaactttgaggacttcttcagcaagatcgtcgcctttcttaccacggacgcgaccctggtggcggcaggtcaggcttggcaggcgctgcgcgtccgccgggacaacatcgacacgtacaccaccagcctcccggactccttcacgggtaacggtcggaaacaaatccacacattccgctatgatccgcggtcgcttaacataaacaaccccgcccagaacggttcggagtccttctggtacaccaactcgggcttctccgccgggagcagctacggtcaatggaaactgcgacaggcgcgcgaagtcaagaccgtgcgcatcaaggcccccatcgggaccagctacgcgagctatgcccccaagtccttccggctccaatactcggatgacggaaccgcttggactacggccctgaccgtctcgaacgcgccgaactggtccgccggggagcagcgggacttcgccgtgcctggcacccccggttcgcacctgtattggaagatcatttgggacgctacccaggtggtgagctacatagggtggcaggaactcctcctgctcgaagcggacgggacggtggccaaccactttgggtcggaggtcatcctaaaggccctgggcaactcgggtctggatgaaatctacaccggcatccgggcggagtatgacagcgccgcaggctggtacaacctgttcatgaacgggtacactggctatgacgccaacgaaatgtcttggtttaaccaaccgggagccctcccgggatacggggcgcaatacactcgggcaaccccgatggtgccgctgtggaacaccaccatgccgtactggatggtggcttcgggccgctccttccggttctgcgtcaaggtcggtacgaactatgaggggggctatcttggtttcattctcccgtatgctacgcccaatcaatacccgtacccgctcgctgtcggtggttccctctgccccgtcaacgacagctcccggtccgcggagtggcgttattcatacgtgagcttcgcccacggcgtgtatcccgggccgggcactcagaactacccggaaagcgaagcgaactgggcgaccctttacctgcgcagcccggaaggagcctggaactaccacggcaaccgttctgcttacgcttcgtccaacagcgagggcgtagggggtccgaccgttagcagctcgcctccctacaacgtcgtcattaacaacgccggtttgcgcaacgtctggcctcactgcatgaacggccagtggtcctcgggccttcgcccctaccgcgagtgcttgggcggcgggtatattctccagccttgcgtgctgattcagcggtcgcctgcccaagtcctcggggagctggaggggacgtttgcaatcagcggctaccaaaacagcgcggagaacacgaccgtgttcaacggcaagactcacgtggtgttccagaatgcttaccgcaacacgatccacgagcactgggcgctgtcgatggattgagggagaactgaatcatggcttatgaaactgggtccgcgaccggaccgaacgacatgttgatcaagctgcgcgacttcgccgcggcccagggttggaccgtgaaccgggacgcggcggcgggctccgggcgcgagttgtgtctgagcaagggggcgtcctacgtcaatttgcgcagctaccagaacgaaacgatcatcatcaacggctcctccacctccgggcgatacgggatcgccatcaacggttcggacggctacagcgccggggcgacttgggaccgccagcccggctatccgctgtgcacttcgtcctcgggcggggaccaggcgcatgccaatcttccgctgcccatctacttcgggccgtttccgtcataccacttgtttgcgccggacagcaagaccatctacctggagctggaggtggcatccactatcttccagcgtctgggtttcggagccctggacttgtttaactccgcggccccgggcggggggcggttcttctacgccaccgggggctcgcacccggcaactactaccggaagcgccacttggctgggatcggacgtggagaactggagctattctctggaggaggtccccttcagggcggcagattacacgacctcctcaagtaccctttccgggtccttcctccgggcgcagttcgactccttcaacaactggtgtcactcctcgcgcagcccgaccaacacccaaaccggacaggcttgccaaggtggggcgattcacgataaagtattgatgtcgatgtctcccaaccccctgaacggggtcgggattctcctgcctcagatcgtgtctgtcaaccgcaacgaggagtacctgaacccggtcggagtcatgcctggtctgcgctatatggacatgaccctgtaccagccgggggaggagttcacgctggggtcggagacgtggaaagtgtttccgtggtaccagaagggcgggcggtccgtccaacggggaatcgcatacaagaaggtgacttgatatggcagtgatcaccacgcaagccttcgtggggctggataccctgcgagccccgacccctgattgggcggtcgggctggattcctatgcgtgggacgatcaaagcccgcccggaaagccatgggagcgaaccgcggacggcttcggctccgtccagaacaacctccccatcagcgaagccggggaggtttcgacgggctggcgcatgccgacctttctggacgactactacaaccgcatccatatccgcccctcgaacatcaacgtgggcaacctcgtgagtgagcagcagttcgcaatcgaggtgtggaacggctttttcaacagccgacaactccagaatatccaagttcagaacggcggcggtatttcccttgtgggggccgtcccgcccgcgacttgggcagctctggagaccaagacctatcagctgaccgtcaccacggacggaccacccgacatcaacgccatcttccattttgattgggatgggacggctgatgacggcgacctccgcgtgctgggctcgcgtatcgtcgccttgccgtacatcttcgaggcccccgccaaggaggtcctggagtggaaaacggacgtgctcacgaccaatgacgggtcggagcagcgggtgcgcctgcgcaagaagccccgccagtccttcaacgtcacctatccgatcccgtaccgggaaatggcccgggcggagaacctggtgtatggttggttgactcgccgttgggccgtcgccctctggtctgaggcccaacaggtcggaaccctgctggcgggcacgaccgtgatcaacatcgacacgaccgcctccgactaccgggacggcgcgctgatcatgatctgggagtccaaccgcaagagcgcgaccgctgacgtggggatcgtttccgccggggctttgacgctgaaccgaccgctggccgaaaccttcaacaacccctggatcgtgcccgtgcgccttgggcggatcgtcggcaacgtctcgcgggcaacctcgggctacaacggttcactggaaatgacctatgagttcagcgacaacatcgacctggacccgcccgcggctcccacgcagttcctcggatatgatgtgtattttgacgaggctctgaagaatggcgaggcgctgacggacagccttcaagcccgggttgatgtcgtggactacgggaccgcggcgggggccagcttctattcgccctggacctacacgcgaattggacgcccctacaagttcttgctacagggactccaggacatctggaacttccgcaagttccttcaccggcgtgcgggacgcctgcgcccgttctgggtcccaaccttcgagaacaacatgcgtgtcgcccagaccggcgagctgacccagagcatcgaggtgtatgctgacgactaccgcgaatttgcgccggagcgcactcacatcggcatcctcctggatgacggaacgtggttgctgcggacgatcaacgcggcgacggcctccgggacggacacggcggtgatcggtctggacgccccgatcaacatcaacgccaatcgcatccgccaaatcagcttcctgggcctgaagcgcctggacgcggatcgggtagaacttcagtggaactccaaccgggtccttgaatgtacggtccgcatgatggagattcaaccatgacgtatgacgcacgcgagcgaagcctgtttgaagcctacccggtcgagctgtacctgttcgcccggggcgcgcaatactggcgctacacctcagcggatgaagacaaggtggtggacggagtgacttacaactccgtccagatcaagcgcggggccttcgagcagaaccaggaaatgtcccggagcaacctgacgctgacgatggataagggcatcagcttccttaaccaattccgcggatcgccgcccaccgacatcgtccaactcaccattcagcggtatcacgagggtgacggacagctcgccgtcccgtgggtcgggcgagtggtgaacgtcaaattcacggagcgcgaggcggaggtgcgccttgagccggtatacacctccctgcgccgcccgaccctgcgccggatgtaccaaacaacttgtccccacgtcctgtacggggccgcgtgcggcctgtcctccgcgaacttccgggtggacgcgaccctcacgggcgtctcggggcgggacctcctgtcaccggccttctcctccttcgctgacggctacttcgccgggggctacgtggattgggaagtggccggggtcctggaacggcggttcatcgtcgcgcacgtggggcaggcgatcaccctcaatcttccgttggccggaatacccgccaacgcgacggtccgggcctatcccgggtgcgaccacaccttgaatacgtgtcacaacaagttcagtaacgtggacaactacgggggtcagccgttctacccgaagaagaacccgatgaacggcaccccgatcttttgaggaggaccccatcatggagtgggctgtatatctgatcatcttcatcgtcgcggcatacgcggcggtggccctcgccccgaagcaggccacccccaaacccgcttcgttggaggacttccaattcccaaccgcggagcccgggcgaccgatcccggttgtgttcgggaccgttaccgtgaagagcccgaacgtggtatggtacggggacttggccagcagtcccgtcaaaacggctggtggcaagtgatgaacaacgagccagtgatggtccgggtcgaacacgcccgcgccttgggctactgctcccgcggcatgcgcgccttcgccgcccgacacgggctggattggggccgcttcgtccacgagggcatcccggcggaggagctggaggcgaccggcgatcacatggcgctacaagtagtggagaaggcccgtgggcagcaaatctagtgtaacaattgggtacaagtattaccttggcgcccacctcgtgatctgtcacgggccggtcgattccgtccaggaaattgtcgtgggcgaccgaaccgcctggagcgggaacgtgactgcctcacagcaaatctacgtcaacaacccggagttgttcggtggcgagaagaaggaggggggtgtccagggttacgtggacatcatgatgggggaatcgaatcagggccgcaacagttacctccagtccaaactcggcacggtcatacccgctttccggggcgtcctgtccctggtccttcggaaggtgtacatgtgcgccatgtcgccctatccgaaggcttgggcgctgaaggtgaagcgcctcccgggcaaggcttggtacccggagaaggcggacatcaacggctccgcgaaccctgcccacgtcatctatgagacgctgacgaacccggactgggggatgggatacccgatcaacgccctggatgacgccgcctttcgcgctgcggcggacacccttcacgcggaaggcttgggcgtgtcgatgatcatgaccaagcaggactccatcgagtccttcatatacacggtgctgggccactgtaatggaatgctgtacacgcgacccgacaatggtcaattcgtggtgaagctgatccgcgaggactacgtggtggcggacctcccgctgttcaacgagtccaacacgatccggctggagtccttcgagcgcccgggctacgcggaaattgttaatgagatcgtggtgacctaccgcccgcaaggctccactgaggacgattccgtgaccgtccaggacctcgcggcgattcaagcacagcagggggtggtgagtcagacggtgaactatccggggattgacaccgcggcgaacgcggcgaagctggccatgcgcgacctccgccagaagtccaccccgttcgcgcgcatccgcatccgggtgaaccggaacgcatggaacctgaccctgggggacgtgttccgcttctcctgggatgagcacaacctcgtggacatcgtgttccgcgtcctcggggtgaactacggggagctgaccagcggcgaaatcgtggtggacgcggttgaggacatgtttggccttccgtcctccacctacatgggcaaccagggctcgggatgggtggacccggttcaagcgcccaacccgttcgccctccgccgtctggaggaggcgaactattgggacttggcgaacggtctgccctcgggcgacttccaggcgctggacaacacctccgccttcctgatcggcctgatgggcgagcccgcccagtacctccagaactatgaactgtggacgaagcccacgggcgggtcctacgcatacgcggccaccggcgaccccgcggcgcacgctacgctgacgaacgcgatcacgcccatacagacctccatccagctgtccaatctgtcctcccgcaccgaatttgcgcggacggggacctatgcgctgattgacaacgaaatcgtgcgcgtggacactatcgacctggtgaacgggatcgtgacggtgggtcgggggtgcttggataccgtctgcgcggaacacgcagccggggcgcggttttggttcgcggaggacgcccgcgtgcgcgaccgtcttgagtacaacagcggcgagaccatcgccgcgaagggcctgggccggtccggggtcggcattctggacctgtccgttgcgccggaggactcgaaggcactggtgggccgtttcgcacgcccctacgctcccgggaacttccgggtgaacagtctccagtatccttcggctatcctcggaggtctgagcctatcttgggcgcaccgcgaccggacccagcaggtggtccgtccgatcatcgaccactccgcggcgaacatcggcccggagccgggggtgacctaccgcgtggacatctacgcggccaacggcagcacgctcctgaagtcggagccgggcctgaccggcactagctggacctggaccaacgaggcgacggagaacaccgcgggccggaaccggatcaaggtcacggcggtccgcgacggcctggacagctaccaatcccacgattggtatgtggatcgggccggactcgggaacaatcttggaaattatcttggaggtttgtgatggctatcagtaacggcccgaacttgggcatcatggtgaacggcgcgctgggggaccagcactacaaccaattcatgtctttcctccgggcggtggacggccttctcatgggccacgcgaagtccgcgaccacgaccgcccaaccggcttcgcccgcggacggggacgtgtacgtgctcccggcgagcccgaccggcacgaactggtctggtcagggccaacggatcgcgcgctattcgagcgcggcgacggcctgggagttcttcgtgccgaagaaggggtggaccatttccgtggaggataccaacagcacctactggtatgacggcagcgcgtggaagttcctccgcggctacggcacgaccgcgaaccgcccggcggcgagcgccgccctgatcgggggccaatacttcgacaccaccctgggcaagccgatatggtccacgggctccgcctgggtggacgcgactgggttggccgtctaaaatttgccaagttgtcttgggtcccgtagaatacggcccaagatcatcttggtgcgaggaccccgatatgcccctgaccccggagcaagtcgaagacatcgccgttgcggctgcgacccgggcggcgaaactatccgtggaggacgcggcgaagcgagccgcggaaacggttgccatgtctcactcggagctgaacgacgtagtggccgaagcggtcaagcagacgttgatgcagctcggggtggacacgtccgacccgttcgccatgcagagggacttccaacacctccgccagtggcgcgagtccggggaggacctgaagcggaaggggaccgttgccctgctgggcatcttcttctccggtctggtctccctgatcctcctgggcctcaaggagtggttccaaaaatgagaatgcgcttgggctacttaccttcacacctgaagaagtatagaccccaagcgccatcgaaagcccagcgccgtaacagctccgaccctcctgcgcttaggttacttcactttctccagttcagttctacttcgcccgataaatcgcccggaccccctgcccagggaggcgaccggcgaccgttcctgctgttcggaggccgtccgggggtttaaggtaagtaagttaagtaagttaagaagaagaagaagaagaatatataaacccccagccccgctgggcttccctgcttactccacttcatacttcttcagcacacgaagtcgagcgttgggcccccgtcccaagcgcacatgattctccgctcgccttcgccgcccagctgggctatacttccgggcatcactatgagaaatggagccaccctatggaataccccttcaagaccgaacccttcaaccaccagcgtgaggagtggttgcgctcccgcgaagaagaagcccgcgcgatcttctgggaacagggcaccggcaagtccaagctgaccatcgacaccgcctgctggctctggctccgcgggctcatcgacggcgtgctggtggtcgccccgaacggcgtgcaccgcaactgggttgagaaggaaatcccggaccacgtacccgatgaggtgatcaagcacgtccgggccttccactaccagagcccgaaggccgacaccaagtggcacaagcaggcggtcaaggccgtcattgagcacaagggcttcgcctggctcaccatcagctatgaagccttcatgaccgcctccgggaagcgggcgctgattgacttcttcgacaagcgccgcctcctgtacgtcctggatgaggcgcactacatcaagaccccgaccgcggagcgcaccaagtccatcctccgctccgcgaagtacgcgccattcaggcgggtcctgaccgggactccgattgctcagggacccttcgacgcctacagccagatcaagttcttgattgacgactactggaacaagaaccagctggggaccttcacggagttcaagcagcacttcggcatctggaagaagggctggaacccgaccgccttcaaccccaagaccaagaagaacgatggcaacgagtatgacgtgctggtgggctatcgccgcctggacgccctgaacagcctccttcagcccgtctcctcccgcgtgacgaaggatgacgtgctggacctcccgccgaagctgtacagcaagcggttcttcccgatgaccccggagcagggcaagctgtatcgccagttgcgtgacgagtacatcgtgtggctggagacgggcgggattgagcgggacgcggaagcggtcgccgcggagccgtcgccggacgcctgcccgacctgcttgggcaaacgtgaggtggagtttgacggcttcatctacccctgccccgactgcggagacgcccctgacctgggcgcggagggcaccaccccggtcatcgccgccctcgccatcacccggctcctccgcctccagcagatcacctgcggctacctcccgaccgacgatgaagcggaacccgtgtacacaatcccggggccgaaccgtcgcctggacctgctctgtgagctgatcgaggagtcccagcacaaggtgatcgtctgggcccggttccagatggacatcaccctgatcatggacgccctccgcgagcgcggcatcagcgcggtccgctatgacgggctggtgaacgatgatgagcgggcggacgccaaggcccggttccagggcgagcgccccctgtaccacaacggacaggtggttgggcgcgaggccgtcccgccggaggagcaggcccgcgtgttcgtgggcaaccccgcggcgggggcgacgggtctgaccttgaccgcagccaagactgtcatttattattccaacagcttcaagctgattgaccgcctccagtcggaggaccgcgcccaccggatcggacagaccaacaacgtgctgtacatcgacctcgtggcggaggactccgtggatgagaaggtggttgaggctttgaggaacaaattcaacgtggcgagccagatcaccggcgaccgcctcaaagactggttgtgagactactatgagccgtgtatttgttgtacagaaccaacaccgctgggaccgcgacaagcagcggttcgagcccaaatttgatctgaccccggcggaggagttcggtgagctggtgtacttgctcagcccgaccgcggcccccttccgcccggagccgatcattgatgagctgaaggagaagctggccgacttcgggccgggggaccacctcctgctcgtgggcaatccggtcctgatcgggttcgccgtcgccatcgccgcggacgccaatgatggggacgtgtccctgctccagtggagcggcaaggaccaacgctacatcgcggtggacgcctcgggcctctttacttcttccgattgaccggctatacttcttcagcgtgattgggataccccctcaccgaagaaacggagaaccacatgtcaagtgaaaacgcatacctggactatgtccaacctcagaccgccggtggcgaactgagccaactcactcagctggccgaacaacaggccgctgcccagtcgaaggtcgcagacctcgaagcccagctcaacaaggcccgcgaagaactccgcgacatcgcggagcgccaggtgcccgaactcatggaccagatcggcattggcgagttcaagaccaccaccggcctgaagatcaagattgacgagacgatccgcgccagcatcccgaaggccaaggccccgctcgccttcgcctggctcaagcagcacggccacgccgcgatgatcaagcgcgtggtcgccgtcgccttcggcaagggcgaggacgagaaggctgacgaactgcgccagcgtctcgcggacgagttcgaggtggacgacaacgccagcgtccatccttcgacccttgccgctttcgtccgcgagaagctgcgtgaaggcgaggaagtccccctggacctgttcggggtccatcgtcagcgcgtgtccaagatcgaagtgtgaccagaatgccggaggacggccccgggccttcctcccgaccgaaccgccccgcgggtgacagcgggtacagccggtgagacggcagggctattcgaccgggggcccaatcgacccgctcacattgaaccgaaggagccacaccatggccaagaccgatagcaagaccaccgatgtcgcagtgaaggaacagaacaccgcaatggcggagtatggcgcatatgccgactacgcgggcgcgggtttcgagaaccagaccagcgatgactacagcatcccgttcctccagattcttcaggccctcagcccgcagctccaggagaacgacagcctgcgccagggcatgatcctgaacaccgtgaccggcgaagtctgggacggcaagaagggcattgccttcgtcccggcgaccacccagcacgtgtacgtggagtggaagccccgcgatgcgggcggcggtttcgtgggcatccacgaagtcaacagcgatctggtgaaccacgccaaggccgcgtcctcggagtatggcaagtacagcaccccggacggcaacgagctgatcgaaaccttctatgtgtacggcatcgcgctggatgatgacggcaacgcctcggaagcggtcctggccttcagctccacgaagatcaagaagtacaagggctggatgaccaaggccaagaccatccagattccgctgccggacggtcgccgcattccggctccgctgttcgcccaccgctaccgcctcaagaccgtgagcgagaagaacaacaagggccagttcttcaactgggacgccatcgccttcgacggcgagaacgcccaacaggctcgcctcctgcccgatgacccgctgttccagtccgccgtgaacatcaagtcgatgatcgagcagggcaaggcccgcgctgcctatgagtcgcaggctccgggctccgcggacgaagaagcccagggcgcaggcggcggcaagccggtgttctgatctaccgggaggaccgacccggacggcccgccccctcgggccgtaccttcagggggccttcgtggcccccttcttttcatcagaaacggagaacgatcatcatgtggagtccgcaacagcagaccgcgctggaccgggttgggcggtggctcaagacccgggacaagcccgtgttccagctcgccgggtacgccggaaccggcaagaccaccctggccaaacacctcgccgcgaccgtcaacggtcccgtgtacttcgccgcctacaccggcaaggccgctcacgtcctcacgaagtccggggcgaccaacgtgagcaccatccacaagctcatctacacgcccaaggacaagtcgcagcagcgcctgaaggaactccaagcggagcgggcgaagctgctaacccacaagcccgtcccggaaaccctcgtggagaaggtcgatgcggcgatcaaggcggagcagatcaacctcgcccgcccgatgttccagctcaacacggagtcgcccctgttcgaggccgcgctgctcgtggtggatgagtattccatgattgacgagcagatgggggaggacttgctcagcttcggttgcccgatcctcgccctgggcgatcccggacagctcccgcccgtgggcggcacccccttcttcaagaacaagcccgacatcctgctcacggagattcaccgccaggcccaggacaacccgatcatctggatgtccaaggaggtccgcgagggccgcgtgctccgccccggcgactacggcgccagccgcgtgattccctatggccgcctgccgcgcgaagaactccgggacatggtactgtccactgaccagctcctcgttggcaggaacgccacgagaatcacgagcaacggacgtgcccgtgaactcctcgggcggacgaacgccctgccgcaggaaggcgacaagctggtgtgcctccgcaacaaccacgaggtgggcctgctcaacggtcagctctggaaggtccgccgtgacacgatcttcgacggcgactatgtcatcatggacatcgaaggcgaggacggcgcgaaggtcgaagtcagcgcccacccccactacttccacggcagcaagccggagtattgggagcggaaggacgcggaggagttcgactatggctatgcgctcaccgtccacaagtcgcagggctcccagtggaacaacgtcctgctgtttgatgagtggtacgggaaggaccggaaggaatggttgtacaccgccattacccgggccgcggaacgcatcgacctcgttatgatgtagcccaagaacaggagcaacgatatgatagaaagccctcaacccttcaaggagactcgcaaaatgcacggtcctcaagtaccctactcacaagaactacacgcccagaagtaccgcggcagcggcgagtccttccgcgaggccatgaaccggatcgccgcggccctgaaggacgatgaccagcacttcgcggacttccgggacgccctcctgggcatgcgcttcctcccggcgggccgcatccagtccgcgatgggctccacccgccaagtcacaccctacaactgctatgtctccgggacgatcaacgacagcttcgtggacggcgaaggctccatcatggtccgggccgcggaagccgcagccacgatgcggatgggcggcgggatcggctatgacttcagcaccctccgtcctcgcggcgacctgatccgcaagctccagtcccactcctccggccccatcagcttcatgcacatcttcgacgcgatctgcaagtgcgtcgcctcctccggccatcgccgcggagcccagatgggggtgatgcgcgtggaccatcccgacatcgaggagttcattcacgccaagcaacccgggaaggacgttcagccgctctgggacctcgtggccgaactcccggagggagcccagaagcagcagttggtcatgtcccttcagcagaccctgaagctgaccggcttcaacgtctccgtcgccatcaccgacaagttcatggagtgcgtcgcctccggcgagccgttccccctcaccttcgagggccggacctaccgcgaagtggacgcccgggcgctgtgggacgcgatcatgcgcgggacctgggattgggcggagcccggggtgctgttcatcgacgcgatcaaccgcatgaacaacctctggtactgcgagaccatcgccgccacgaacccctgcggtgagcaaccgctcccgccctacggtgcctgcttgttgggctccttcaacctggtcaagtacatcttcaaggacggggcgggccgctacgccttcgactgggaccagtaccgcgaggacatcccgcaggtggtccgcgcgatggacaacgtggttgatcgcgcgatctacccgctgccgcagcagaagcaggaagccaaggacaagcgccgcatgggcctcgggatcaccggcctggccaacgctgccgaagccctgggccatgagtacggttcgcccgccttcctcgccttcgaggcggaggtgctggacacgctgcgtgatgagtcctacctggccagcgcccacatcgccaaggtcaagggctccttcccgaagttcgacaaggacaagtacctccagggccagttcatcaagaccctccgcgaggacgtgcgggacgccatcgccaaatacggcatccgcaactcccacctcacttccatcgccccgaccgggaccatcagcctgtgcgccgacaacgtcagctccgggattgagccggtgttcgcctacagcttcgaccgcaccgtgatcgagttcagcggcccgcgggtggagacggtggaggactacggtgcccgcgtgttcggggttcgcggcaaggcctgctcccgcgtcaccgtccaggaacacgtcgccgccctgaccgtcgccgcccagcgggtcgattccgcggtgagcaagacctgcaacgtgccttccgacatcagctgggaggacttcaagaacgtgtacgtgagcgcctgggaaggcggggcgaaaggctgcaccaccttccgtctgggcgggaagcggtcgggcatcctcgtggtgaaggatgacggcggcgagcccgaagcggacgccccggcggaggagccggcaagccagtgccgcatcgacccggccacgggacggagggagtgcgagtgaaagaactgagcctgaaggcggtcttgctgatcgccgccgggttcttgctcatgaccgggatgcgccttgctgaatgggccatcccggtcccggagcggaccctcaaactgaacgtcacccaagaaatggaggaacccgaagatgaacaagcccctgctgatcggtcaagcacccggacctaacacggacccggaccggcccctggctcccctcccgcggtcctccgcgggagggcgtctggcggagctggcgggcctatcgcccaaggactacctcaagaccttcgaccgcaccaacctgctccacaccttcccggggcgctggaagcgggacgacaagtggcccgcccgggacgcggggattgccgcagccgcgatgaagcccttgttgggcggtcggcacgtcatcctcgttgggcggaacgtcgcagaggctttcggctatccggcccagcacctggacttccaccagtggtttgcggatgatcgctggggcttcgaggtcgctgtggttccgcacacctcggggcgcaaccattggtacaggaagcctgggcacgaggacgccgcccgggccttctgggaagaagttgtacaacggttcgccctccgccgtccaacggttgttggccttcggacggggacctgaaaaagtttagtcaaaccactttacttcttcgggggctggggttaagattctctcacggtcgaacaagatcgcacctcaaccccagaaaaggagcctaccatgaacgccatcaacttcaacaacgtcgcctacaccgaagcctccctgagcgagctgtccggcccggccctggtcgagctgtacaacgaagtcatcggcaccttccgcaacggcgagtccgtcccgaacgtccgccgctttgccgacaagaccaccgccattgcccgcacctggaagatgcttcagcgttatgccgaagcgcacccggaagttgaggctgacgagcaggccgaaccccagaaggtcgaaaccgtgaacgaaaccgcaacccccgcccccgtcgctgctccgaaggcccagaaggctccgaagtccgcggaggagaagaaggcccgcgccccgcgcggcaccaacctggccgccccgggccacgccccgatcccctgccgcgagggctcgaagcaggccatgctcctggacatgctgtcccgcccgaacggtgcgaccatggctgaactgatcgaagccctgagtggcggcaacaagccctggaccgaagccaccgtgcgctccggcttcggttgggacatgaagctgaagggctacggggtccgctccgccttcgccgcggacggcactgagcggttccacatcgtggtccctgaaggccacgcgatcccggcccacaagccgctgaagtccgccccgaaggctgacgcccgccagacccgcctggttggctgaggcaagggtcatgggagcctcggagcgcacctatgactacctgatccgccgggtggagtacccggcggagcggggatacagaatggagcccttcaagctacctccgtggattcacgtggtgatcacggaggacggcgacagcaagtggctgacggtccattcccgtattcacgtcaacaaagaagtccgcatggagccttccttcagtcgccaattctctgattgggacatcttgaaggacctgagcgggaaaatcagtcacgcatacttgtgagaaaagattatgagcagaaactacccccggctggacatcgagacgtttggccgacatctgatcaccaccggcgatctggaccccatctacacggccctggttcgggcggagcaggcgggggacttctccgtgccgcagctctgtcgttggctccttggatattggtgctactaccacgccggggtcgcctccttcctgagtgagaaggagggcgaggagttctggcactggatgatggtcgcggcccgcaacgaggaggagacgcccgccggaggacgctggccccggggacacgagcgccgccactaccgggccaagatcgccgtggactccgtgacctccctccaggcccgctacggcgaccgcccggagaacatggccctgtacgtgggagcccgggcgacggaggatgagcgcctgcccttccgcaccgtctccgcccgcgcccaggagcacaacggcttcggtccgtggatcggcttcaagatcgcggacatgatggaccgggtgatggaggtcccggtggacttcgacaacgccgccgtgttcatgttcaaggacccggagaaggccgcgatgatgctgtgggagcagcgcgaggcgcacaagtacccggagaacgcgaagccgaagcgcgaggcgatcctgtccggggtcgcggactacctgattgggcggttcgcggacctcgccgccccgcccctgggcgaccgccccgtgaacatccaggaggtcgagacggtcctgtgtaaatggaagtcccacatgaatggccactacccgctctggaacgacatccgggaaatcaacggcgggctcgaaccgtgggcgggccgctgctccgccgcgcgggccttcctcaaccacatgcccaaggagcagtgagatgatcgtcaacaacaccccggtcgaaacctatgagctcaacggggtcccgatcctcgtgaagcgggaggacctgtgcgccccgctcccgggtccgtccttcagcaagattcgcggagttgtcgcccatatcaagaaccggcctgagaccaccatcggctgtctggacacgtaccactcgaaggcgggctgggcggtcgcctacgtctgccagcagctcgggaaacaggccgtggactactggccccgcttcaagcgcgacggggccgcggacgccccgcgcgtccaacagcagcacgctcgccagctcggggcggacctcgtggacatcccggcgggccgctccgcgatcctgtaccacacggccaagaagcacctgcgggagaactaccacgacagctacctgatgccgaacgccctgaagctcccggagtcgatcacggagaacgccgcggaggccgtccgcaccgccccgcacctcccggactccgggaccctggtcatcagtatcagctcggggacggtcgccgccggggtgctcaagggcttcgaggaggcgggcctgctccgcaactacaacgtcatcctccacatgggatactcgcggagccaggacgccacccgggagtacatcgagaaggccgcgggcctgaccctgggcgaccggatcaagttcattgacgagggctacgggtacgcggacgcggcccgggacgcctccgccccgttcccctgcaacccgttctatgatctgaaggcttggaagtggctgagtgacccgctcaacctggcttccgtccatccacgccccatcgtgttctggaacatcggggagtgacccaattcatagtgctttacttcttccgggtaaggcactagactttttcgcaatagatgaggagttgaactatggaccacgcagcatggctgaatgaagaaaccggcgaagccgctcaggaggcttacaagtatttcatgcgcccggacccgaaccaacgggagttcctgggcccaatcgaggaggaggatgacccgctgaccggcatgcgcgcgaagttccgcatggccaaggtggggatggtccgcaacgcgaaggatgacgacaagaaggaggtcaaggtgtatcttggcttcaatgacgtcacctacctcccgcacatccgcatcccgaacgccaagccccttcagggctggtaccaggacaagcacaacgacaagcgaggctcccgcgcccgcccctgcttcagcgaggcgatcctgacggagccttatgggggctactgcaccgtgggttgcgccttctgctacgtcaacagcgggttccggggctaccgcggcaccggcctcatcagcgtcccggtgaactacggcgagcaggtccgcaacatgctctcgaagtcccggacctccgccgcgggctacttctccagcttcacggaccccttcctgccgattgaggacgtgtaccacaacacccagcagggggcggaagccttcgtggagttgggcctgcccatcttcttcctgagccgtctcagctacccgtcctgggccatcgacctcctgaagcggaacccctacagctacgcccagaagtcgctgaacaccggcaacgaccgcgattggcacaagttgtcccccggggccatttccctccaggaccacattgacgaaatcgcggagctgcgccgtcagggcatctacacgtccattcaggtcaatccggtggtcccggggatcgtcacccatgacgacatccgccacctgttcgagcgcctggccgcggtcggcaacaaccacgtgatcgtgaagttcgtggaagcgggctacagctgggctccggcgatgatcgaacgtctccacaagcggttcggcccggagcgcaccaaagccttcatggacctgttcacggagaaccaggccggagcccaaaagaccatcgcggagccgtaccgggtcgaagcccaccagctgtaccggaagtgggcgacggagctgggcatgacctacgcgacgtgctatgagtaccgccgcgggaagcccggaaccggcgaaccggcctggctttcgatgggccgtgaaatgatcaccgcggaccagtgccacggccagcgcgtcccgatgttcacccggaccgatctgggccagcccttccaggaggtcaaggagtgcgcccccaccggctgtctccactgcgcggacgacaacgagggcaagccccgctgcggttcggaactgttcggggcggcgaaggctctgcgctcgcccgacttcaagaagatcgtggaaccgaccccgccggaggaggacggcggcgagcgcaagatcatcccgatcacgcagattgactgagcaacccgggcggggctccggctccgccgttttcaactgaaatggagaaccaagatgaagtacatcaacgtgcggggctgtaacggctccggcaagaccaccctgctgcgctgcctggcccgcgatccgctttgccgcgtcatcaacgtcatcgtcccggaccacaagccgatcccggtgacgtatgccccggacggcatcgccatcatcggggactacacccccgccgccgccggagcgaccaccgccggtctggaccggatcaagacccaagccgccgccaaggccgtcgcggagctggttgggcgggacccggacgtgaaggcggtcctgttcgagggcgtggtggtcagcaccatctacggtccgtggcaggagtggtcgaaggcgaacggcggaatgatctgggccttcctggacacaccgctcgaagtctgcctgaagcgcatccaggagcgcaacggcgggaagcccatcaaggaggaccaggtggccgacaagcaccgcaccatcgcccgggtccgcgacaaggccctggcggacggcgagacggtccgcgacatccactgggagacggccctgaaggacatcaaggccgtcatcgagaacttgggctgaggaccccgactatgaccacaccgcgcctcaacgacatcgccgccttcatgaaggcccggcacgacatctacttggaccgcaaggccgggaagcccggcccctggaccgcggacccggttctgcgtgatgggcggttctgcaacatcttccgggagctggacacggtgacgatctgggttgacaagcatatccgtcagccctacgcggaccacccgcacctctggttcatgctcgccatcgcccgctacatcaactggccggataccctcgcggagctgatccagaccaagcagtggcccgacaaccctgacttcgagccctcctggctcacgaccgctctggagcatcgcgccgtccgcggcgacaaggtgtacaccggagcctacatgatccgcgcggagtccgacccctccaaggagtggtacagctggaccaagcaccgctacatcgcggagattgtcctgggccgtctctgggaggaccgcgaggaatggcagcggatgctggaaaccactccgggcgtcctccggtccttcaaccggctcgaaaccgtctgggagaagttccagcagcaacgctacatcggctggggtccgttcatggcctatgaggtggtgaccgacctccgccacacccgctacctgcgcaacgccccggacatctgggcttgggccaacgccggtcccggggcgatccgcgggctcaaccgcctgtatgggcgcgacctcgccgcgaagccccgcccggagcagacgaacgcggaaatgatcgagctgatgcaggagctgaacgccctggacgcccggggcttcaacgaaaccttcggaccgccgcagctcgggagcccgcacgtggggccgcggttcgaggcccgggacattgaacacacgctgtgcgagttcgacaagtatgagcgcgtgcgcctgaacgaaggcaagatgcgctcgaagtatgactggcgcaaggcaaccaccctcgcctgatcgaaaccccgccgccggaccattccggcggcaccaacgaaatggagaaaccatcatggctgtacgtctgtccaattacatccgcgagcaggtccgtgacgcgatcctcgcccactccttctccgaccgcgagaaggccctggacgcccgcgagaaggagctggcgctggagttctacaacgacctgtacccggaagcggtccgcgcccacatgtacgccctgcccaacggcttcctcgaagtccgcagcagcatccgcgtccaggtggttggggagtcctaccactcgctggacctcccggagaagaagcgcgtggccgattgctgggcctcgaaccccggcaaggtctataacgcggaccacccgctgggcgagaagctgcgcacctacctgaaggaccgcgcccagttcaagcgcgagcgggaggaggccaagaccggagcctgggccgtcctcgaaagcgtgaccacggtcaacaagctgattcaggtctggccggaggtggagcagttcgcccgccccttcgcggttgaatcgccgtcccgggctatcgcgctgccgatcaaggacctgaacgcccgcctgggccttccgcctcagaccgcttcggcttaacaggagggggccatgatcttctcgccgttctggtggtactggagctggtggttggtctggctccctcgcccccgcgtccttcgccggaccggcaacgtcatcttcgtggagttcaacaagaaatgaaagtcatcaagacccgcaacgtacaacaggccctcccggaggccctgtatcaactgtccttcgagggcgtccgccgcgactcgcgcaacggccccgtgttcatgttcccggaacccgtcaccaccgtgtacctccgcccggcggagcgcgtgctgttctgggcggaacgggacgccaaccccttcttccacctgatggaaagcctctggatgctgggcggacgcaatgacgtggagtacgtcgcccgcttcgtggatcgcatgcgcagctactcggatgacggcctgaccttccacggggcctacggcttccgctggcgccagcacttcttcgaggaccagctgcccaagatcatcgccgccctgaaggcgaaccgcgatgaccgccgccaggtcctgtcgatgtgggacgcggacgcggacctgggccgccaaggcaaggacctcccctgcaaccttcaggccatcttccagatcgcctgtgacggtcgcctggacatgaccgtgaccaaccgctccaacgacctgatctggggagcctacggggccaacgcggtccacttcagctacctccatgagtacgtcgcccggagtgtcggggttgaacaaggcatctaccgccaagtcagcgccaacttccacgcctatgaggaggtgctggacaaggtcgccccgctcgcggaactcgccgccaacccgatgaccgggaaggagacgcccgacccctacgccgccgggatcgcggagccgtacccgctgatgtccacggacccggaggagtggaaccaggagctgatgatgttcctgagcgagccggacgccgtgggcttccgtgacccgttcttccgtcgcgtggcgatcccgatgttgaaggcccacaaggctttcaagcagacctccaacccctcccgctttgacgccgccttggcggagctggacaacgtcgccgccaccgactggaagctggccggggtggagtggatcgaacgccgccgcgccgccttcgaggctcgcaaggcccgggcgatggacgatggcgtggcgtatgagtgaggagacgcaataatgggaagcctgatgagcaagattcatgacgaggagcgcgaggcggaggagctgaaccgccgcgccgcccgcccgctcctgacccggatcgccgcgaccagggaggccgggacggtccgccggtgtcacatcgttccgcaccacggtcagtacaacatcgcccagcacagctacggggccgtgagcctcttgctgctgctccacccgcacccgtcgctgaacctgatcaaggcggtccagtggcacgactgcgcggagcgttggttgggcgacatcccggccccggcgaagtggacccactccgaactcgggaaggtgtatgaggaggcggaacgccgcgtgctggcgaccctgggcctgctcccgggccttctccctgacgaggaggactggttgaaggccgtggacaccctcgaactgtggttgtggtgccgggaggaagaagccctgggcaacgaagcggtcacggccatgcggagggcatgcgaggcggtgacggagaagcggggcctggagggtagcctgcccgaacccgtccgcgccttctacgtggcagcgaagcaccagccgcatggccgtctctcggacttcttcgaggaggtggtgcgcgatggacttggagaagctgcgacgtgattgggcggaggacccgcagctgaagttctacgccttcgacacggtggaagaactcgctgcgcacctccgcaaggtccatacagatatgatgaacggggagcacgggtgttttgggtacttgtaccgccagcagacactccggctccgggaactgatgaaggagttacaagatgagcgtgaacgaaaagcaagtgggcggtgagcactaccgctcgcccgttcaacactgggactacgtggagctgaacggcctccgctacaccgaaggctgcgcgaccaagtacgcgacccgcaaccgcaagaagcacgaggacccgcgccaggaccttgagaaggcgatccactacgtggagaaggtccaggacctgtaccgcaacggggtcctgctgccccgctccgcccccgtggtcattaccccggacgccttcgccgccgcgaacgggctgacggaggacgaagccgaagtggtccgcatcctcaccttctgggagtccgacccggagctgaccgcggccctgaacctcctgcgcaagatgattgaggaggtcggagcctgatgtcatacctccaaccacccctgttcacgaccgtctccagcgactgggtggccccggacctcaacaccctcccctcgtgggagggggccaagcgggtcgccatcgactgcgagacgcgggacccggacctgcgcaaactcggaccgggggcgggccgtcgcccgaacagctacatcaccggcatcagcttcgcaatcgaggacggcccgggcgggtacttgcccatcagacacgaaggcgggggcaacctcccgctggagggcgtgctggcctacctccgcgcccaggcaaaggtgttcaccggcgacctcgtgggggccaacctcccgtatgacctggacttcctcgccggggacggcatcgagttcgagcgggtccgctacttccgtgacatccagatcgctgacccgctgatctgcgaactccacgacagctacagcatgcaagctatcgcggagcggtggggcttccacggcaaggacgaagccctgctgcgcgccgccgcggtcgattatgggattgacccgaagaaggacatgtggatgctcccggccaagtttgtcgggaagtacgcggaggaggacacgcgcctgcctctgaacatcctccgccgtcaggagcgggagattgatgagcaggacctctggggcgtgtacaacctggagtccaagctgctcccgatcctcacgggccttcgccgccggggcgtccgaatcgactgcgaccgcctggacatgattgagcgttgggcgctggagaaggagacggaggccctggcccaagtccggtcgatcaccggccaccggatcgccgtgggcgatgtctggaagccggaggtgatcgcccccgccctcgaacacatcggcatcaagctgaacaagacctcccagggcaagcccaacatcgacaaggagctgctgggctcaatcgaccaccccgtggcggacctcctcgaacgcgcccggaaggtgaacaagctgcgcacgaccttcgccagctccgtccgggaccacatggtgaacggtcgcctccacgggacgttcaaccagctccgccgccagaaggatgacgaaagcgacgggaccgcgggcgctgcctacgggcgactgtccagcgaacacccgaacctccagcagcaaccggctcgggatgagttcgccatgatgtggcgggccatctacctcccggaggaaggccaacactgggcgtccaacgactacagccagcaggagccgcgcatggcggtccactacgcctgcttggcgaaggacctgattgggcaccaagcctggctgtccgcaatcgaagcccgggacaagtaccgcaacgacccgaacaccgacaaccaccagatgatggcggacatggcggggatcaagcgcaaggacgccaaggaaatctacctgggcctgtcctacgggatgggcggggcgaagatgtgccgcaagctcgggctcccgactatgatggccgtgcgcggcccccgcttccagctgttcgacgtgaacagcccggagggtcagcgcctggtcgcggaaggggcgcggaggttcgaggccgcggggccggagggtcaggccctcctggacaccttcgaccacaaggtgccgttcatcaagaagctggcgaaggcttgcgaagcccgggcgaaggccgtgggctacatcacgaccctgagcggtcgccgttgccgcttcccgaaggacaaggacgggaactatgactggacccacaagggactgaaccggctgattcagggctcctccgcggaccagaccaagatggcgatggtggcctgcgcggaagccggactggacatcatcatccaggtccacgatgagatcgccttcagcgtacacgacatgaaggaggccgcggaagccgcccacatcatgaggacgtgcacgccgctcgaactcccgtcaaaggtggacgtggagattgggcagagctggggtcattccatgggctgggacgggaacccaccatcatgaagttctgctatcaatgtgacgcgcaggtcacttacttgtttgcggacgcacgctgcgcaaagtgtacccgcctgaccccggaggaagtccggggcgaacccctggagaacgatatgcgccgcagcaacgacaacaccgtggacctcgaagtggtcatcaagcgcgagacagacaaggcatacctcatcgaccacggcggtgaggaggaagtctggatgcccaagtcacaggtccgcgcggtcgagaagaagggccgcacagcgaccctgacggtcaccgaatggatcgccaacgagaaggggctgatatgaacgacatcgccgtgcgctggacctcccggaagttctgggcggcgatgatctgggaggcggtcctggtttggctcctgtacatgggcaagttgccggtggacgccttcgagtccttgacctggctcctgctgggcggttacttcctcgggaacgtcgcccagaaggttttgctgaaggaggaggtgaaatgagcgaacgtcaagaccgctgggaccgccgctatgttgggctggcccaacacgtcgcgggctggagcaaggacccttccacgaaggtcggagccgtcctggttcggcccaacaacagcgtggcttcgaccgggttcaacggcttcccgcccgggcacgatgattcgccggagctgtacgctgaccgcgggtacaaataccagcacgttgttcacgcagaggtcaacgcactcaactttctgggctcgcctgcgactggcttcacgctctatacttctttcccctgctgtccgaactgtatggaggccgcggggaaggcgggcgtgaagcgggtcgccttcccgggcatcgactactcgggccgcgatccggggtgggttgctgagtggaatcaacgcattgatgaggctttggaagtcgcccgccgttacaacatcgaagtgaggtgggtagatgtctgaagccgcaatgtgggactccctccgccccgtcatccggtcgctggacccggtgcgcgtggagaaccccattgtgcccgggaccccggatgtgaactacaaccagggctggattgaattgaagttcgctgaacgctggccgcccaggggcggaccgcttcgagtggaccacttcacccgccagcagaggacctggctgacccgtcgccgcagggccgggggccgggccttcctcctgctgaaggtcggggagacggagtggttgctattcgatggagcggtggccgctgctatgctgggccgggttccgcgagaacgcctgtatgaggtctgtgtcgcacgttggacacgccttccaagaaccaaggagatttgtacatgtctgctacagtgacaccaaccaaaggcgaaagcctactgctacaccgccgccgcaagggcctcaatcagattgaggccgcgaaggagtacggggtgcacccggaccgctaccgtgaatgggaagcggaccgccgcctggacgatcaaccgcgccagcacctcggacaactgaagccccacgaggtctgcttgctgttccgccgccgctcgggtaagacccagcgcgaaatcgccgccgctctgggctgcactcgcctctgggtcatccagatggaggacgggaaagcgccggttgagcgccttcgtgaatattggggcttttgagggggatcggaaatggcggaactgccgaaacacaagaccaaggacgcaatcgacttcctgaagaagtggtgcccggaggggccgtgggtcctgacggccatcatcccggacgggaaaacggagacggtcacattcatgcccgaccgctggcagaaagccgcggagtggatcgaaggacatcagggcaagcgcaacctgtacttccacgtgaacccggtccgccgggcgatggacgtgaaagcctcgaaggaggacatggcccgcctcgcctggcttcacgtggacatcgacccgcgagccggggaggacttcgaggaggagcgggcgcgggcgctgaagctgctccagtcctacacgcccaagcccacggtcatcatcgactcgggcgggggctatcagggcttttggcgtctgaacccgtccgacaagctggacatcgccggatcggtggcgaaggctcaagagctggaagcctacaacatccagctggagaaggtgtttcaggcggaccactgccacaacgtggaccgcatcatgcgcctcccgggcacgatcaacatgcccaccgcgaagaaggtcaagaagggtcgccagccgaccctcgcccgtctcgtggagtggaatgaggccagctaccccatcgaacaattcacccccgcggttcgagtccagatggcggagcagggcctggccgggggccgtccgaaggtgaagatcacgggcaacgtcccggacatcggaacggaggagctgcgggagtgggcccatgagcacgggaaggctatcagcgaccacgtgctggcgctgattgctactgggcaggacccgctggacccgaccaagtacccctcccggtcggaagccctgttcaaggtctgctgcgacctcgtgcgggcggaggtccctgatgaaatgatcttcgcggtgatcaccggctccaacgaaatcgccgcgagcgtcagagacaagccgaactgggaaggctacgccctgcggcagatcgaacgtgcccacgaggaggcggtggacccttggctgcgcaagctcaacgagaagcacgccgtcatcgcggacatcggcgggaagtgccgcatcatcagcgaggtctgggacccggcgatgaagcggaccaaaatcagcaagcagtccttcgaggacttccgcaaccgctaccgccacatcaaggtagtggttgggcactcggaggagggcaagcccatcgagaaggccgcgggagccttctggattgatcacccccagcgccgccaatatgagaccatcgtgtttgcccccggccaggaggtcgaagaagcctacaacctctggcgcgggttcgcgtgcgactccctcccgggcgagaagcacatgcccttcctgaaccacatccgcgacaacgtctgctcagggaacccggagcactaccactacctggtcgggtggatggcgcggatggtccagcacccggacggcccgggcgaagtggccgtggtcctccgcggtcgccgcggcaccggcaagtccttcttcgccaaggtcctgggcgcgatgttcgggcgtcactacctccaagtcagcgactcgaagcacctggtgggctccttcaacgcccacctccgcgataccgtcctgctgttcggtgatgaggctttcttcgccggggacaagaagcacgaaagcgtgctcaagaccctcgtgaccgaagaacacctggtgatcgagggcaagggcgtggacgcggaagcggccccgaactatgtccacctggtcctcgcctcgaacgaagattgggtggtgcccgcgggtctggatgaacgccggttcttcgtcatggaggtgggtgagggacacaagcaggaccacgcctatttcaagcgcatcaaggacgatctggacaacggaggacttgagcacctgctccacttcctcctgacctatgacctgagcgccttcgaggttcgccaggttccccagacccgggcgctgcaggaccagaagatcatgagcatgtcgccggaaacccagtggatgtatgagaagctgtgggagggccggttgctcaagaccgaccaggactggcggaacaaggtggtgaaggacagcttgtatgacgactacgtgaacgacctccgcgaccagggccggaacttccgcatgagccgcaccggcttcggcaagtggcttgcccgggccttcccggacggctggccgcagtcgaagcaggaaatggcggagattccatggaccaatgaacacggcttcgaggtgatgatcaagaagcgcgtgtacatgtacca

SEQ ID NO: 2 - DNA, 20 bp, synthetic construct
  source 1..20: mol_type = other DNA
gcgcagtcatgagatcgaga

SEQ ID NO: 3 - DNA, 20 bp, synthetic construct
  source 1..20: mol_type = other DNA
gttgagtgcaccgagagtga

SEQ ID NO: 4 - DNA, 20 bp, synthetic construct
  source 1..20: mol_type = other DNA
tgggtcacttcggtgttacg

SEQ ID NO: 5 - DNA, 20 bp, synthetic construct
  source 1..20: mol_type = other DNA
gtggtgaaaggtgcggtttc

SEQ ID NO: 6 - DNA, 20 bp, synthetic construct
  source 1..20: mol_type = other DNA
cgtagtcgcgattgtcggta

SEQ ID NO: 7 - DNA, 20 bp, synthetic construct
  source 1..20: mol_type = other DNA
accactgctgacgttcgatt

SEQ ID NO: 8 - DNA, 20 bp, synthetic construct
  source 1..20: mol_type = other DNA
gctaccggtacgactacgtg

SEQ ID NO: 9 - DNA, 20 bp, synthetic construct
  source 1..20: mol_type = other DNA
gatctggaaacagccgtcca

SEQ ID NO: 10 - DNA, 19 bp, synthetic construct
  source 1..19: mol_type = other DNA
tttcggtggcttggatttt

SEQ ID NO: 11 - DNA, 20 bp, synthetic construct
  source 1..20: mol_type = other DNA
atttgcgagaagtacaactg

SEQ ID NO: 12 - DNA, 20 bp, synthetic construct
  source 1..20: mol_type = other DNA
atcccctttgcatcttcaat

SEQ ID NO: 13 - DNA, 20 bp, synthetic construct
  source 1..20: mol_type = other DNA
ttccgtcatctaagggaatc

SEQ ID NO: 14 - DNA, 20 bp, synthetic construct
  source 1..20: mol_type = other DNA
taagcccttcgtaaagttct

SEQ ID NO: 15 - DNA, 20 bp, synthetic construct
  source 1..20: mol_type = other DNA
aagcattgaaaaacgaaacg

SEQ ID NO: 16 - DNA, 21 bp, synthetic construct
  source 1..21: mol_type = other DNA
actaggagaagattagatggc

SEQ ID NO: 17 - DNA, 16 bp, synthetic construct
  source 1..16: mol_type = other DNA
ctggtccgtaagggtg

SEQ ID NO: 18 - DNA, 20 bp, synthetic construct
  source 1..20: mol_type = other DNA
gatatacgagcaacgtcttc

SEQ ID NO: 19 - DNA, 20 bp, synthetic construct
  source 1..20: mol_type = other DNA
atttgcgagaagtacaactg

SEQ ID NO: 20 - DNA, 20 bp, synthetic construct
  source 1..20: mol_type = other DNA
gttattgcgacggttaaaga

SEQ ID NO: 21 - DNA, 20 bp, synthetic construct
  source 1..20: mol_type = other DNA
tggattaaatactacgccga

SEQ ID NO: 22 - DNA, 20 bp, synthetic construct
  source 1..20: mol_type = other DNA
ctggcaaaacaacctcatta

SEQ ID NO: 23 - DNA, 20 bp, synthetic construct
  source 1..20: mol_type = other DNA
agttaccacgaggatttcat

SEQ ID NO: 24 - DNA, 19 bp, synthetic construct
  source 1..19: mol_type = other DNA
gtagatgttcggttcggta

SEQ ID NO: 25 - DNA, 20 bp, synthetic construct
  source 1..20: mol_type = other DNA
caagccaattcacatcgtag

SEQ ID NO: 26 - DNA, 20 bp, synthetic construct
  source 1..20: mol_type = other DNA
attctgtttcaacaaccctg

SEQ ID NO: 27 - DNA, 20 bp, synthetic construct
  source 1..20: mol_type = other DNA
cagacatccaggaacttttc

SEQ ID NO: 28 - DNA, 20 bp, synthetic construct
  source 1..20: mol_type = other DNA
catacctacgatatacggca

SEQ ID NO: 29 - DNA, 20 bp, synthetic construct
  source 1..20: mol_type = other DNA
gactactcgctctacatcaa

SEQ ID NO: 30 - DNA, 20 bp, synthetic construct
  source 1..20: mol_type = other DNA
atggcctttcttcattcttg

SEQ ID NO: 31 - DNA, 20 bp, synthetic construct
  source 1..20: mol_type = other DNA
agaaaatatccgggtgtgat

SEQ ID NO: 32 - DNA, 20 bp, synthetic construct
  source 1..20: mol_type = other DNA
tagattgtgattcacgcaac

SEQ ID NO: 33 - DNA, 20 bp, synthetic construct
  source 1..20: mol_type = other DNA
gaagacgaaaaggcaaaaac

SEQ ID NO: 34 - DNA, 20 bp, synthetic construct
  source 1..20: mol_type = other DNA
atattgaactccgaagtcgt

SEQ ID NO: 35 - DNA, 19 bp, synthetic construct
  source 1..19: mol_type = other DNA
ctaccaaactgggggatag